European Patent Specification EP 3 223 848 B1, published November 27, 2024. Title: METHODS OF USING BISPECIFIC ANTIGEN-BINDING CONSTRUCTS TARGETING HER2. Applicant: ZYMEWORKS INC. Application NOT YET ASSIGNED. The sequence listing filed with the application follows.

SEQUENCE LISTING (350 sequences)

SEQ ID NO: 1 - protein, 450 aa, Artificial Sequence
  Description of Artificial Sequence: Synthetic polypeptide
EVQLVESGGGLVQPGGSLRLSCAASGFNIKDTYIHWVRQAPGKGLEWVARIYPTNGYTRYADSVKGRFTISADTSKNTAYLQMNSLRAEDTAVYYCSRWGGDGFYAMDYWGQGTLVTVSSASTKGPSVFPLAPSSKSTSGGTAALGCLVKDYFPEPVTVSWNSGALTSGVHTFPAVLQSSGLYSLSSVVTVPSSSLGTQTYICNVNHKPSNTKVDKKVEPKSCDKTHTCPPCPAPELLGGPSVFLFPPKPKDTLMISRTPEVTCVVVDVSHEDPEVKFNWYVDGVEVHNAKTKPREEQYNSTYRVVSVLTVLHQDWLNGKEYKCKVSNKALPAPIEKTISKAKGQPREPQVYTLPPSRDELTKNQVSLTCLVKGFYPSDIAVEWESNGQPENNYKTTPPVLDSDGSFFLYSKLTVDKSRWQQGNVFSCSVMHEALHNHYTQKSLSLSPGK

SEQ ID NO: 2 - DNA, 1350 bp, Artificial Sequence
  Description of Artificial Sequence: Synthetic polynucleotide
gaggtgcagctggtggaaagcggaggaggactggtgcagccaggaggatctctgcgactgagttgcgccgcttcaggattcaacatcaaggacacctacattcactgggtgcgacaggctccaggaaaaggactggagtgggtggctcgaatctatcccactaatggatacacccggtatgccgactccgtgaaggggaggtttactattagcgccgatacatccaaaaacactgcttacctgcagatgaacagcctgcgagccgaagataccgctgtgtactattgcagtcgatggggaggagacggattctacgctatggattattggggacaggggaccctggtgacagtgagctccgcctctaccaagggccccagtgtgtttcccctggctccttctagtaaatccacctctggagggacagccgctctgggatgtctggtgaaggactatttccccgagcctgtgaccgtgagttggaactcaggcgccctgacaagcggagtgcacacttttcctgctgtgctgcagtcaagcgggctgtactccctgtcctctgtggtgacagtgccaagttcaagcctgggcacacagacttatatctgcaacgtgaatcataagccctcaaatacaaaagtggacaagaaagtggagcccaagagctgtgataagacccacacctgccctccctgtccagctccagaactgctgggaggacctagcgtgttcctgtttccccctaagccaaaagacactctgatgatttccaggactcccgaggtgacctgcgtggtggtggacgtgtctcacgaggaccccgaagtgaagttcaactggtacgtggatggcgtggaagtgcataatgctaagacaaaaccaagagaggaacagtacaactccacttatcgcgtcgtgagcgtgctgaccgtgctgcaccaggactggctgaacgggaaggagtataagtgcaaagtcagtaataaggccctgcctgctccaatcgaaaaaaccatctctaaggccaaaggccagccaagggagccccaggtgtacacactgccacccagcagagacgaactgaccaagaaccaggtgtccctgacatgtctggtgaaaggcttctatcctagtgatattgctgtggagtgggaatcaaatggacagccagagaacaattacaagaccacacctccagtgctggacagcgatggcagcttcttcctgtattccaagctgacagtggataaatctcgatggcagcaggggaacgtgtttagttgttcagtgatgcatgaagccctgcacaatcattacactcagaagagcctgtccctgtctcccggcaaa

SEQ ID NO: 3 - protein, 120 aa, Artificial Sequence [sequence omitted]

SEQ ID NO: 4 - DNA, 360 bp, Artificial Sequence
  Description of Artificial Sequence: Synthetic polynucleotide
gaggtgcagctggtggaaagcggaggaggactggtgcagccaggaggatctctgcgactgagttgcgccgcttcaggattcaacatcaaggacacctacattcactgggtgcgacaggctccaggaaaaggactggagtgggtggctcgaatctatcccactaatggatacacccggtatgccgactccgtgaaggggaggtttactattagcgccgatacatccaaaaacactgcttacctgcagatgaacagcctgcgagccgaagataccgctgtgtactattgcagtcgatggggaggagacggattctacgctatggattattggggacaggggaccctggtgacagtgagctcc

SEQ ID NO: 5 - protein, 8 aa, Artificial Sequence
  Description of Artificial Sequence: Synthetic peptide
GFNIKDTY

SEQ ID NO: 6 - DNA, 24 bp, Artificial Sequence
  Description of Artificial Sequence: Synthetic oligonucleotide
ggattcaacatcaaggacacctac

SEQ ID NO: 7 - protein, 13 aa, Artificial Sequence
  Description of Artificial Sequence: Synthetic peptide
SRWGGDGFYAMDY

SEQ ID NO: 8 - DNA, 39 bp, Artificial Sequence
  Description of Artificial Sequence: Synthetic oligonucleotide
agtcgatggggaggagacggattctacgctatggattat

SEQ ID NO: 9 - protein, 8 aa, Artificial Sequence
  Description of Artificial Sequence: Synthetic peptide
IYPTNGYT

SEQ ID NO: 10 - DNA, 24 bp, Artificial Sequence
  Description of Artificial Sequence: Synthetic oligonucleotide
atctatcccactaatggatacacc

SEQ ID NO: 11 - protein, 98 aa, Artificial Sequence
  Description of Artificial Sequence: Synthetic polypeptide
ASTKGPSVFPLAPSSKSTSGGTAALGCLVKDYFPEPVTVSWNSGALTSGVHTFPAVLQSSGLYSLSSVVTVPSSSLGTQTYICNVNHKPSNTKVDKKV

SEQ ID NO: 12 - DNA, 294 bp, Artificial Sequence
  Description of Artificial Sequence: Synthetic polynucleotide
gcctctaccaagggccccagtgtgtttcccctggctccttctagtaaatccacctctggagggacagccgctctgggatgtctggtgaaggactatttccccgagcctgtgaccgtgagttggaactcaggcgccctgacaagcggagtgcacacttttcctgctgtgctgcagtcaagcgggctgtactccctgtcctctgtggtgacagtgccaagttcaagcctgggcacacagacttatatctgcaacgtgaatcataagccctcaaatacaaaagtggacaagaaagtg

SEQ ID NO: 13 - protein, 110 aa, Artificial Sequence
  Description of Artificial Sequence: Synthetic polypeptide
APELLGGPSVFLFPPKPKDTLMISRTPEVTCVVVDVSHEDPEVKFNWYVDGVEVHNAKTKPREEQYNSTYRVVSVLTVLHQDWLNGKEYKCKVSNKALPAPIEKTISKAK

SEQ ID NO: 14 - DNA, 330 bp, Artificial Sequence
  Description of Artificial Sequence: Synthetic polynucleotide
gctccagaactgctgggaggacctagcgtgttcctgtttccccctaagccaaaagacactctgatgatttccaggactcccgaggtgacctgcgtggtggtggacgtgtctcacgaggaccccgaagtgaagttcaactggtacgtggatggcgtggaagtgcataatgctaagacaaaaccaagagaggaacagtacaactccacttatcgcgtcgtgagcgtgctgaccgtgctgcaccaggactggctgaacgggaaggagtataagtgcaaagtcagtaataaggccctgcctgctccaatcgaaaaaaccatctctaaggccaaa

SEQ ID NO: 15 - protein, 106 aa, Artificial Sequence [sequence omitted]

SEQ ID NO: 16 - DNA, 318 bp, Artificial Sequence
  Description of Artificial Sequence: Synthetic polynucleotide
ggccagccaagggagccccaggtgtacacactgccacccagcagagacgaactgaccaagaaccaggtgtccctgacatgtctggtgaaaggcttctatcctagtgatattgctgtggagtgggaatcaaatggacagccagagaacaattacaagaccacacctccagtgctggacagcgatggcagcttcttcctgtattccaagctgacagtggataaatctcgatggcagcaggggaacgtgtttagttgttcagtgatgcatgaagccctgcacaatcattacactcagaagagcctgtccctgtctcccggc

SEQ ID NO: 17 - protein, 448 aa, Artificial Sequence
  Description of Artificial Sequence: Synthetic polypeptide
EVQLVESGGGLVQPGGSLRLSCAASGFTFTDYTMDWVRQAPGKGLEWVADVNPNSGGSIYNQRFKGRFTLSVDRSKNTLYLQMNSLRAEDTAVYYCARNLGPSFYFDYWGQGTLVTVSSASTKGPSVFPLAPSSKSTSGGTAALGCLVKGYFPEPVTVSWNSGALTSGVHTFPAVLKSSGLYSLSSVVTVPSSSLGTQTYICNVNHKPSNTKVDKKVEPKSCDKTHTCPPCPAPELLGGPSVFLFPPKPKDTLMISRTPEVTCVVVDVSHEDPEVKFNWYVDGVEVHNAKTKPREEQYNSTYRVVSVLTVLHQDWLNGKEYKCKVSNKALPAPIEKTISKAKGQPREPQVYVLPPSRDELTKNQVSLLCLVKGFYPSDIAVEWESNGQPENNYLTWPPVLDSDGSFFLYSKLTVDKSRWQQGNVFSCSVMHEALHNHYTQKSLSLSPG

SEQ ID NO: 18 - DNA, 1344 bp, Artificial Sequence
  Description of Artificial Sequence: Synthetic polynucleotide
gaagtgcagctggtcgaatctggaggaggactggtgcagccaggagggtccctgcgcctgtcttgcgccgctagtggcttcacttttaccgactacaccatggattgggtgcgacaggcacctggaaagggcctggagtgggtcgccgatgtgaacccaaatagcggaggctccatctacaaccagcggttcaagggccggttcaccctgtcagtggaccggagcaaaaacaccctgtatctgcagatgaatagcctgcgagccgaagatactgctgtgtactattgcgcccggaatctggggccctccttctactttgactattgggggcagggaactctggtcaccgtgagctccgcctccaccaagggaccttctgtgttcccactggctccctctagtaaatccacatctgggggaactgcagccctgggctgtctggtgaagggctacttcccagagcccgtcacagtgtcttggaacagtggcgctctgacttctggggtccacacctttcctgcagtgctgaagtcaagcgggctgtacagcctgtcctctgtggtcaccgtgccaagttcaagcctgggaacacagacttatatctgcaacgtgaatcacaagccatccaatacaaaagtcgacaagaaagtggaacccaagtcttgtgataaaacccatacatgccccccttgtcctgcaccagagctgctgggaggaccaagcgtgttcctgtttccacccaagcctaaagatacactgatgattagtaggaccccagaagtcacatgcgtggtcgtggacgtgagccacgaggaccccgaagtcaagtttaactggtacgtggacggcgtcgaggtgcataatgccaagactaaacccagggaggaacagtacaacagtacctatcgcgtcgtgtcagtcctgacagtgctgcatcaggattggctgaacgggaaagagtataagtgcaaagtgagcaataaggctctgcccgcacctatcgagaaaacaatttccaaggcaaaaggacagcctagagaaccacaggtgtacgtgctgcctccatcaagggatgagctgacaaagaaccaggtcagcctgctgtgtctggtgaaaggattctatccctctgacattgctgtggagtgggaaagtaatggccagcctgagaacaattacctgacctggccccctgtgctggactcagatggcagcttctttctgtatagcaagctgaccgtcgacaaatcccggtggcagcaggggaatgtgtttagttgttcagtcatgcacgaggcactgcacaaccattacacccagaagtcactgtcactgtcaccaggg

SEQ ID NO: 19 - protein, 119 aa, Artificial Sequence [sequence omitted]

SEQ ID NO: 20 - DNA, 357 bp, Artificial Sequence
  Description of Artificial Sequence: Synthetic polynucleotide
gaagtgcagctggtcgaatctggaggaggactggtgcagccaggagggtccctgcgcctgtcttgcgccgctagtggcttcacttttaccgactacaccatggattgggtgcgacaggcacctggaaagggcctggagtgggtcgccgatgtgaacccaaatagcggaggctccatctacaaccagcggttcaagggccggttcaccctgtcagtggaccggagcaaaaacaccctgtatctgcagatgaatagcctgcgagccgaagatactgctgtgtactattgcgcccggaatctggggccctccttctactttgactattgggggcagggaactctggtcaccgtgagctcc

SEQ ID NO: 21 - protein, 8 aa, Artificial Sequence
  Description of Artificial Sequence: Synthetic peptide
GFTFTDYT

SEQ ID NO: 22 - DNA, 24 bp, Artificial Sequence
  Description of Artificial Sequence: Synthetic oligonucleotide
ggcttcacttttaccgactacacc

SEQ ID NO: 23 - protein, 12 aa, Artificial Sequence
  Description of Artificial Sequence: Synthetic peptide
ARNLGPSFYFDY

SEQ ID NO: 24 - DNA, 36 bp, Artificial Sequence
  Description of Artificial Sequence: Synthetic oligonucleotide
gcccggaatctggggccctccttctactttgactat

SEQ ID NO: 25 - protein, 8 aa, Artificial Sequence
  Description of Artificial Sequence: Synthetic peptide
VNPNSGGS

SEQ ID NO: 26 - DNA, 24 bp, Artificial Sequence
  Description of Artificial Sequence: Synthetic oligonucleotide
gtgaacccaaatagcggaggctcc

SEQ ID NO: 27 - protein, 98 aa, Artificial Sequence
  Description of Artificial Sequence: Synthetic polypeptide
ASTKGPSVFPLAPSSKSTSGGTAALGCLVKGYFPEPVTVSWNSGALTSGVHTFPAVLKSSGLYSLSSVVTVPSSSLGTQTYICNVNHKPSNTKVDKKV

SEQ ID NO: 28 - DNA, 294 bp, Artificial Sequence
  Description of Artificial Sequence: Synthetic polynucleotide
gcctccaccaagggaccttctgtgttcccactggctccctctagtaaatccacatctgggggaactgcagccctgggctgtctggtgaagggctacttcccagagcccgtcacagtgtcttggaacagtggcgctctgacttctggggtccacacctttcctgcagtgctgaagtcaagcgggctgtacagcctgtcctctgtggtcaccgtgccaagttcaagcctgggaacacagacttatatctgcaacgtgaatcacaagccatccaatacaaaagtcgacaagaaagtg

SEQ ID NO: 29 - protein, 110 aa, Artificial Sequence; identical to SEQ ID NO: 13
  Description of Artificial Sequence: Synthetic polypeptide

SEQ ID NO: 30 - DNA, 330 bp, Artificial Sequence
  Description of Artificial Sequence: Synthetic polynucleotide
gcaccagagctgctgggaggaccaagcgtgttcctgtttccacccaagcctaaagatacactgatgattagtaggaccccagaagtcacatgcgtggtcgtggacgtgagccacgaggaccccgaagtcaagtttaactggtacgtggacggcgtcgaggtgcataatgccaagactaaacccagggaggaacagtacaacagtacctatcgcgtcgtgtcagtcctgacagtgctgcatcaggattggctgaacgggaaagagtataagtgcaaagtgagcaataaggctctgcccgcacctatcgagaaaacaatttccaaggcaaaa

SEQ ID NO: 31 - protein, 106 aa, Artificial Sequence
  Description of Artificial Sequence: Synthetic polypeptide
GQPREPQVYVLPPSRDELTKNQVSLLCLVKGFYPSDIAVEWESNGQPENNYLTWPPVLDSDGSFFLYSKLTVDKSRWQQGNVFSCSVMHEALHNHYTQKSLSLSPG

SEQ ID NO: 32 - DNA, 318 bp, Artificial Sequence
  Description of Artificial Sequence: Synthetic polynucleotide
ggacagcctagagaaccacaggtgtacgtgctgcctccatcaagggatgagctgacaaagaaccaggtcagcctgctgtgtctggtgaaaggattctatccctctgacattgctgtggagtgggaaagtaatggccagcctgagaacaattacctgacctggccccctgtgctggactcagatggcagcttctttctgtatagcaagctgaccgtcgacaaatcccggtggcagcaggggaatgtgtttagttgttcagtcatgcacgaggcactgcacaaccattacacccagaagtcactgtcactgtcaccaggg

SEQ ID NO: 33 - protein, 214 aa, Artificial Sequence
  Description of Artificial Sequence: Synthetic polypeptide
DIQMTQSPSSLSASVGDRVTITCKASQDVSIGVAWYQQKPGKAPKLLIYSASYRYTGVPSRFSGSGSGTDFTLTISSLQPEDFATYYCQQYYIYPYTFGQGTKVEIKRTVAAPSVFIFPPSDEQLKSGTASVVCLLNNFYPREAKVQWKVDNALQSGNSQESVTEQDSKDSTYSLSSTLTLSKADYEKHKVYACEVTHQGLSSPVTKSFNRGEC

SEQ ID NO: 34 - DNA, 642 bp, Artificial Sequence
  Description of Artificial Sequence: Synthetic polynucleotide
gatattcagatgacccagtccccaagctccctgagtgcctcagtgggcgaccgagtcaccatcacatgcaaggcttcccaggatgtgtctattggagtcgcatggtaccagcagaagccaggcaaagcacccaagctgctgatctatagcgcctcctaccggtataccggcgtgccctctagattctctggcagtgggtcaggaacagactttactctgaccatctctagtctgcagcctgaggatttcgctacctactattgccagcagtactatatctacccatatacctttggccaggggacaaaagtggagatcaagaggactgtggccgctccctccgtcttcatttttcccccttctgacgaacagctgaaaagtggcacagccagcgtggtctgtctgctgaacaatttctaccctcgcgaagccaaagtgcagtggaaggtcgataacgctctgcagagcggcaacagccaggagtctgtgactgaacaggacagtaaagattcaacctatagcctgtcaagcacactgactctgagcaaggcagactacgagaagcacaaagtgtatgcctgcgaagtcacacatcaggggctgtcctctcctgtgactaagagctttaacagaggagagtgt

SEQ ID NO: 35 - protein, 107 aa, Artificial Sequence [sequence omitted]

SEQ ID NO: 36 - DNA, 321 bp, Artificial Sequence
  Description of Artificial Sequence: Synthetic polynucleotide
gatattcagatgacccagtccccaagctccctgagtgcctcagtgggcgaccgagtcaccatcacatgcaaggcttcccaggatgtgtctattggagtcgcatggtaccagcagaagccaggcaaagcacccaagctgctgatctatagcgcctcctaccggtataccggcgtgccctctagattctctggcagtgggtcaggaacagactttactctgaccatctctagtctgcagcctgaggatttcgctacctactattgccagcagtactatatctacccatatacctttggccaggggacaaaagtggagatcaag

SEQ ID NO: 37 - protein, 6 aa, Artificial Sequence
  Description of Artificial Sequence: Synthetic peptide
QDVSIG

SEQ ID NO: 38 - DNA, 18 bp, Artificial Sequence
  Description of Artificial Sequence: Synthetic oligonucleotide
caggatgtgtctattgga

SEQ ID NO: 39 - protein, 9 aa, Artificial Sequence
  Description of Artificial Sequence: Synthetic peptide
QQYYIYPYT

SEQ ID NO: 40 - DNA, 27 bp, Artificial Sequence
  Description of Artificial Sequence: Synthetic oligonucleotide
cagcagtactatatctacccatatacc

SEQ ID NO: 41 - protein, 3 aa, Artificial Sequence
  Description of Artificial Sequence: Synthetic peptide
SAS

SEQ ID NO: 42 - DNA, 9 bp, Artificial Sequence
  Description of Artificial Sequence: Synthetic oligonucleotide
agcgcctcc

SEQ ID NO: 43 - protein, 107 aa, Artificial Sequence [sequence omitted]

SEQ ID NO: 44 - DNA, 321 bp, Artificial Sequence
  Description of Artificial Sequence: Synthetic polynucleotide
aggactgtggccgctccctccgtcttcatttttcccccttctgacgaacagctgaaaagtggcacagccagcgtggtctgtctgctgaacaatttctaccctcgcgaagccaaagtgcagtggaaggtcgataacgctctgcagagcggcaacagccaggagtctgtgactgaacaggacagtaaagattcaacctatagcctgtcaagcacactgactctgagcaaggcagactacgagaagcacaaagtgtatgcctgcgaagtcacacatcaggggctgtcctctcctgtgactaagagctttaacagaggagagtgt

SEQ ID NO: 45 - protein, 222 aa, Artificial Sequence
  Description of Artificial Sequence: Synthetic polypeptide
DYKDDDDKDIQMTQSPSSLSASVGDRVTITCRASQDVNTAVAWYQQKPGKAPKLLIYSASFLYSGVPSRFSGSRSGTDFTLTISSLQPEDFATYYCQQHYTTPPTFGQGTKVEIKRTVAAPSVFIFPPSDERLKSGTASVVCLLNNFYPREAKVQWKVDNALQSGNSQESVTEQDSKDSTYSLSSTLTLSKADYEKHKVYACEVTHQGLSSPVTKSFNRGEC

SEQ ID NO: 46 - DNA, 666 bp, Artificial Sequence
  Description of Artificial Sequence: Synthetic polynucleotide
gactacaaagacgacgatgacaaagatatccagatgacccagtcccctagctccctgtccgcttctgtgggcgatagggtcactattacctgccgcgcatctcaggacgtgaacaccgcagtcgcctggtaccagcagaagcctgggaaagctccaaagctgctgatctacagtgcatcattcctgtattcaggagtgcccagccggtttagcggcagcagatctggcaccgatttcacactgactatttctagtctgcagcctgaggactttgccacatactattgccagcagcactataccacaccccctactttcggccaggggaccaaagtggagatcaagcgaactgtggccgctccaagtgtcttcatttttccacccagcgatgaaagactgaagtccggcacagcttctgtggtctgtctgctgaacaatttttaccccagagaggccaaagtgcagtggaaggtcgacaacgctctgcagagtggcaacagccaggagagcgtgacagaacaggattccaaagactctacttatagtctgtcaagcaccctgacactgagcaaggcagactacgaaaagcataaagtgtatgcctgtgaggtcacacatcaggggctgtcatcaccagtcaccaaatcattcaatcggggggagtgc

SEQ ID NO: 47 - protein, 107 aa, Artificial Sequence [sequence omitted]

SEQ ID NO: 48 - DNA, 321 bp, Artificial Sequence
  Description of Artificial Sequence: Synthetic polynucleotide
gatatccagatgacccagtcccctagctccctgtccgcttctgtgggcgatagggtcactattacctgccgcgcatctcaggacgtgaacaccgcagtcgcctggtaccagcagaagcctgggaaagctccaaagctgctgatctacagtgcatcattcctgtattcaggagtgcccagccggtttagcggcagcagatctggcaccgatttcacactgactatttctagtctgcagcctgaggactttgccacatactattgccagcagcactataccacaccccctactttcggccaggggaccaaagtggagatcaag

SEQ ID NO: 49 - protein, 6 aa, Artificial Sequence
  Description of Artificial Sequence: Synthetic peptide
QDVNTA

SEQ ID NO: 50 - DNA, 18 bp, Artificial Sequence
  Description of Artificial Sequence: Synthetic oligonucleotide
caggacgtgaacaccgca

SEQ ID NO: 51 - protein, 9 aa, Artificial Sequence
  Description of Artificial Sequence: Synthetic peptide
QQHYTTPPT

SEQ ID NO: 52 - DNA, 27 bp, Artificial Sequence
  Description of Artificial Sequence: Synthetic oligonucleotide
cagcagcactataccacaccccctact

SEQ ID NO: 53 - protein, 3 aa, Artificial Sequence
  Description of Artificial Sequence: Synthetic peptide
SAS

SEQ ID NO: 54 - DNA, 9 bp, Artificial Sequence
  Description of Artificial Sequence: Synthetic oligonucleotide
agtgcatca

SEQ ID NO: 55 - protein, 107 aa, Artificial Sequence
  Description of Artificial Sequence: Synthetic polypeptide
RTVAAPSVFIFPPSDERLKSGTASVVCLLNNFYPREAKVQWKVDNALQSGNSQESVTEQDSKDSTYSLSSTLTLSKADYEKHKVYACEVTHQGLSSPVTKSFNRGEC

SEQ ID NO: 56 - DNA, 321 bp, Artificial Sequence
  Description of Artificial Sequence: Synthetic polynucleotide
cgaactgtggccgctccaagtgtcttcatttttccacccagcgatgaaagactgaagtccggcacagcttctgtggtctgtctgctgaacaatttttaccccagagaggccaaagtgcagtggaaggtcgacaacgctctgcagagtggcaacagccaggagagcgtgacagaacaggattccaaagactctacttatagtctgtcaagcaccctgacactgagcaaggcagactacgaaaagcataaagtgtatgcctgtgaggtcacacatcaggggctgtcatcaccagtcaccaaatcattcaatcggggggagtgc

SEQ ID NO: 57 - protein, 222 aa, Artificial Sequence
  Description of Artificial Sequence: Synthetic polypeptide
DYKDDDDKDIQMTQSPSSLSASVGDRVTITCRASQDVNTAVAWYQQKPGKAPKLLIYSASFLYSGVPSRFSGSRSGTDFTLTISSLQPEDFATYYCQQHYTTPPTFGQGTKVEIKRTVAAPSVFIFPPSDERLKSGTASVVCLLNNFYPREAKVQWKVDNALQSGNSKESVTEQDSKDSTYSLSSRLTLSKADYEKHKVYACEVTHQGLSSPVTKSFNRGEC

SEQ ID NO: 58 - DNA, 666 bp, Artificial Sequence
  Description of Artificial Sequence: Synthetic polynucleotide
gactacaaagacgacgatgacaaagatatccagatgacccagtcccctagctccctgtccgcttctgtgggcgatagggtcactattacctgccgcgcatctcaggacgtgaacaccgcagtcgcctggtaccagcagaagcctgggaaagctccaaagctgctgatctacagtgcatcattcctgtattcaggagtgcccagccggtttagcggcagcagatctggcaccgatttcacactgactatttctagtctgcagcctgaggactttgccacatactattgccagcagcactataccacaccccctactttcggccaggggaccaaagtggagatcaagcgaactgtggccgctccaagtgtcttcatttttccacccagcgatgaaagactgaagtccggcacagcttctgtggtctgtctgctgaacaatttttaccccagagaggccaaagtgcagtggaaggtcgacaacgctctgcagagtggcaacagcaaggagagcgtgacagaacaggattccaaagactctacttatagtctgtcaagcagactgacactgagcaaggcagactacgaaaagcataaagtgtatgcctgtgaggtcacacatcaggggctgtcatcaccagtcaccaaatcattcaatcggggggagtgc

SEQ ID NO: 59 - protein, 107 aa, Artificial Sequence [sequence omitted]

SEQ ID NO: 60 - DNA, 321 bp, Artificial Sequence; identical to SEQ ID NO: 48
  Description of Artificial Sequence: Synthetic polynucleotide

SEQ ID NO: 61 - protein, 6 aa, Artificial Sequence
  Description of Artificial Sequence: Synthetic peptide
QDVNTA

SEQ ID NO: 62 - DNA, 18 bp, Artificial Sequence
  Description of Artificial Sequence: Synthetic oligonucleotide
caggacgtgaacaccgca

SEQ ID NO: 63 - protein, 9 aa, Artificial Sequence
  Description of Artificial Sequence: Synthetic peptide
QQHYTTPPT

SEQ ID NO: 64 - DNA, 27 bp, Artificial Sequence
  Description of Artificial Sequence: Synthetic oligonucleotide
cagcagcactataccacaccccctact

SEQ ID NO: 65 - protein, 3 aa, Artificial Sequence
  Description of Artificial Sequence: Synthetic peptide
SAS

SEQ ID NO: 66 - DNA, 9 bp, Artificial Sequence
  Description of Artificial Sequence: Synthetic oligonucleotide
agtgcatca

SEQ ID NO: 67 - protein, 107 aa, Artificial Sequence
  Description of Artificial Sequence: Synthetic polypeptide
RTVAAPSVFIFPPSDERLKSGTASVVCLLNNFYPREAKVQWKVDNALQSGNSKESVTEQDSKDSTYSLSSRLTLSKADYEKHKVYACEVTHQGLSSPVTKSFNRGEC

SEQ ID NO: 68 - DNA, 321 bp, Artificial Sequence
  Description of Artificial Sequence: Synthetic polynucleotide
cgaactgtggccgctccaagtgtcttcatttttccacccagcgatgaaagactgaagtccggcacagcttctgtggtctgtctgctgaacaatttttaccccagagaggccaaagtgcagtggaaggtcgacaacgctctgcagagtggcaacagcaaggagagcgtgacagaacaggattccaaagactctacttatagtctgtcaagcagactgacactgagcaaggcagactacgaaaagcataaagtgtatgcctgtgaggtcacacatcaggggctgtcatcaccagtcaccaaatcattcaatcggggggagtgc

SEQ ID NO: 69 - protein, 214 aa, Artificial Sequence
  Description of Artificial Sequence: Synthetic polypeptide
DIQMTQSPSSLSASVGDRVTITCKASQDVSIGVAWYQQKPGKAPKLLIYSASYRYTGVPSRFSGSGSGTDFTLTISSLQPEDFATYYCQQYYIYPATFGQGTKVEIKRTVAAPSVFIFPPSDEQLKSGTASVVCLLNNFYPREAKVQWKVDNALQSGNSQESVTEQDSKDSTYSLSSTLTLSKADYEKHKVYACEVTHQGLSSPVTKSFNRGEC

SEQ ID NO: 70 - DNA, 642 bp, Artificial Sequence
  Description of Artificial Sequence: Synthetic polynucleotide
gatattcagatgacccagtccccaagctccctgagtgcctcagtgggcgaccgagtcaccatcacatgcaaggcttcccaggatgtgtctattggagtcgcatggtaccagcagaagccaggcaaagcacccaagctgctgatctatagcgcctcctaccggtataccggcgtgccctctagattctctggcagtgggtcaggaacagactttactctgaccatctctagtctgcagcctgaggatttcgctacctactattgccagcagtactatatctacccagccacctttggccaggggacaaaagtggagatcaagaggactgtggccgctccctccgtcttcatttttcccccttctgacgaacagctgaaaagtggcacagccagcgtggtctgtctgctgaacaatttctaccctcgcgaagccaaagtgcagtggaaggtcgataacgctctgcagagcggcaacagccaggagtctgtgactgaacaggacagtaaagattcaacctatagcctgtcaagcacactgactctgagcaaggcagactacgagaagcacaaagtgtatgcctgcgaagtcacacatcaggggctgtcctctcctgtgactaagagctttaacagaggagagtgt

SEQ ID NO: 71 - protein, 107 aa, Artificial Sequence
  Description of Artificial Sequence: Synthetic polypeptide
DIQMTQSPSSLSASVGDRVTITCKASQDVSIGVAWYQQKPGKAPKLLIYSASYRYTGVPSRFSGSGSGTDFTLTISSLQPEDFATYYCQQYYIYPATFGQGTKVEIK

SEQ ID NO: 72 - DNA, 321 bp, Artificial Sequence
  Description of Artificial Sequence: Synthetic polynucleotide
gatattcagatgacccagtccccaagctccctgagtgcctcagtgggcgaccgagtcaccatcacatgcaaggcttcccaggatgtgtctattggagtcgcatggtaccagcagaagccaggcaaagcacccaagctgctgatctatagcgcctcctaccggtataccggcgtgccctctagattctctggcagtgggtcaggaacagactttactctgaccatctctagtctgcagcctgaggatttcgctacctactattgccagcagtactatatctacccagccacctttggccaggggacaaaagtggagatcaag

SEQ ID NO: 73 - protein, 6 aa, Artificial Sequence
  Description of Artificial Sequence: Synthetic peptide
QDVSIG

SEQ ID NO: 74 - DNA, 18 bp, Artificial Sequence
  Description of Artificial Sequence: Synthetic oligonucleotide
caggatgtgtctattgga

SEQ ID NO: 75 - protein, 9 aa, Artificial Sequence
  Description of Artificial Sequence: Synthetic peptide
QQYYIYPAT

SEQ ID NO: 76 - DNA, 27 bp, Artificial Sequence
  Description of Artificial Sequence: Synthetic oligonucleotide
cagcagtactatatctacccagccacc

SEQ ID NO: 77 - protein, 3 aa, Artificial Sequence
  Description of Artificial Sequence: Synthetic peptide
SAS

SEQ ID NO: 78 - DNA, 9 bp, Artificial Sequence
  Description of Artificial Sequence: Synthetic oligonucleotide
agcgcctcc

SEQ ID NO: 79 - protein, 107 aa, Artificial Sequence [sequence omitted]

SEQ ID NO: 80 - DNA, 321 bp, Artificial Sequence; identical to SEQ ID NO: 44
  Description of Artificial Sequence: Synthetic polynucleotide

SEQ ID NO: 81 - protein, 449 aa, Artificial Sequence
  Description of Artificial Sequence: Synthetic polypeptide
EVQLVESGGGLVQPGGSLRLSCAASGFNIKDTYIHWVRQAPGKGLEWVARIYPTNGYTRYADSVKGRFTISADTSKNTAYLQMNSLRAEDTAVYYCSRWGGDGFYAMDYWGQGTLVTVSSASTKGPSVFPLAPSSKSTSGGTAALGCEVTDYFPEPVTVSWNSGALTSGVHTFPAVLQSSGLYSLSSVVTVPSSSLGTQTYICNVNHKPSNTKVDKKVEPKSCDKTHTCPPCPAPELLGGPSVFLFPPKPKDTLMISRTPEVTCVVVDVSHEDPEVKFNWYVDGVEVHNAKTKPREEQYNSTYRVVSVLTVLHQDWLNGKEYKCKVSNKALPAPIEKTISKAKGQPREPQVYVYPPSRDELTKNQVSLTCLVKGFYPSDIAVEWESNGQPENNYKTTPPVLDSDGSFALVSKLTVDKSRWQQGNVFSCSVMHEALHNHYTQKSLSLSPG

SEQ ID NO: 82 - DNA, 1347 bp, Artificial Sequence
  Description of Artificial Sequence: Synthetic polynucleotide
gaggtgcagctggtcgaaagcggaggaggactggtgcagccaggagggtcactgcgactgagctgcgcagcttccggcttcaacatcaaggacacctacattcactgggtccgccaggctcctggaaaaggcctggagtgggtggcacgaatctatccaactaatggatacacccggtatgccgactccgtgaagggccggttcaccatttctgcagatacaagtaaaaacactgcctacctgcagatgaacagcctgcgagccgaagatacagccgtgtactattgcagccgatggggaggcgacggcttctacgctatggattattgggggcagggaaccctggtcacagtgagctccgcatcaacaaaggggcctagcgtgtttccactggccccctctagtaaatccacctctgggggaacagcagccctgggatgtgaggtgaccgactacttcccagagcccgtcactgtgagctggaactccggcgccctgacatctggggtccatacttttcctgctgtgctgcagtcaagcggcctgtacagcctgtcctctgtggtcactgtgccaagttcaagcctggggactcagacctatatctgcaacgtgaatcacaagccatccaataccaaagtcgacaagaaagtggaacccaagtcttgtgataaaacacatacttgccccccttgtcctgcaccagagctgctgggaggaccaagcgtgttcctgtttccacccaagcctaaagacaccctgatgattagtaggactccagaagtcacctgcgtggtcgtggacgtgagccacgaggaccccgaagtcaagttcaactggtacgtggatggcgtcgaggtgcataatgccaagacaaaacccagggaggaacagtacaactccacttatcgcgtcgtgtctgtcctgaccgtgctgcaccaggactggctgaacggcaaggagtataagtgcaaagtgagcaataaggctctgcccgcacctatcgagaaaacaatttccaaggctaaagggcagcctagagaaccacaggtgtacgtgtaccctccatctagggacgagctgaccaagaaccaggtcagtctgacatgtctggtgaaagggttctatcccagcgatatcgcagtggagtgggaatccaatggacagcctgagaacaattacaagaccacaccccctgtgctggactctgatggaagtttcgccctggtgagtaagctgaccgtcgataaatcacggtggcagcagggcaacgtgttcagctgttcagtgatgcacgaagcactgcacaaccactacacccagaaaagcctgtccctgtcccccggc

SEQ ID NO: 83 - protein, 120 aa, Artificial Sequence [sequence omitted]

SEQ ID NO: 84 - DNA, 360 bp, Artificial Sequence
  Description of Artificial Sequence: Synthetic polynucleotide
gaggtgcagctggtcgaaagcggaggaggactggtgcagccaggagggtcactgcgactgagctgcgcagcttccggcttcaacatcaaggacacctacattcactgggtccgccaggctcctggaaaaggcctggagtgggtggcacgaatctatccaactaatggatacacccggtatgccgactccgtgaagggccggttcaccatttctgcagatacaagtaaaaacactgcctacctgcagatgaacagcctgcgagccgaagatacagccgtgtactattgcagccgatggggaggcgacggcttctacgctatggattattgggggcagggaaccctggtcacagtgagctcc

SEQ ID NO: 85 - protein, 8 aa, Artificial Sequence
  Description of Artificial Sequence: Synthetic peptide
GFNIKDTY

SEQ ID NO: 86 - DNA, 24 bp, Artificial Sequence
  Description of Artificial Sequence: Synthetic oligonucleotide
ggcttcaacatcaaggacacctac

SEQ ID NO: 87 - protein, 13 aa, Artificial Sequence
  Description of Artificial Sequence: Synthetic peptide
SRWGGDGFYAMDY

SEQ ID NO: 88 - DNA, 39 bp, Artificial Sequence
  Description of Artificial Sequence: Synthetic oligonucleotide
agccgatggggaggcgacggcttctacgctatggattat

SEQ ID NO: 89 - protein, 8 aa, Artificial Sequence
  Description of Artificial Sequence: Synthetic peptide
IYPTNGYT

SEQ ID NO: 90 - DNA, 24 bp, Artificial Sequence
  Description of Artificial Sequence: Synthetic oligonucleotide
atctatccaactaatggatacacc

SEQ ID NO: 91 - protein, 98 aa, Artificial Sequence
  Description of Artificial Sequence: Synthetic polypeptide
ASTKGPSVFPLAPSSKSTSGGTAALGCEVTDYFPEPVTVSWNSGALTSGVHTFPAVLQSSGLYSLSSVVTVPSSSLGTQTYICNVNHKPSNTKVDKKV

SEQ ID NO: 92 - DNA, 294 bp, Artificial Sequence
  Description of Artificial Sequence: Synthetic polynucleotide
gcatcaacaaaggggcctagcgtgtttccactggccccctctagtaaatccacctctgggggaacagcagccctgggatgtgaggtgaccgactacttcccagagcccgtcactgtgagctggaactccggcgccctgacatctggggtccatacttttcctgctgtgctgcagtcaagcggcctgtacagcctgtcctctgtggtcactgtgccaagttcaagcctggggactcagacctatatctgcaacgtgaatcacaagccatccaataccaaagtcgacaagaaagtg

SEQ ID NO: 93 - protein, 110 aa, Artificial Sequence; identical to SEQ ID NO: 13
  Description of Artificial Sequence: Synthetic polypeptide

SEQ ID NO: 94 - DNA, 330 bp, Artificial Sequence
  Description of Artificial Sequence: Synthetic polynucleotide
gcaccagagctgctgggaggaccaagcgtgttcctgtttccacccaagcctaaagacaccctgatgattagtaggactccagaagtcacctgcgtggtcgtggacgtgagccacgaggaccccgaagtcaagttcaactggtacgtggatggcgtcgaggtgcataatgccaagacaaaacccagggaggaacagtacaactccacttatcgcgtcgtgtctgtcctgaccgtgctgcaccaggactggctgaacggcaaggagtataagtgcaaagtgagcaataaggctctgcccgcacctatcgagaaaacaatttccaaggctaaa

SEQ ID NO: 95 - protein, 106 aa, Artificial Sequence
  Description of Artificial Sequence: Synthetic polypeptide
GQPREPQVYVYPPSRDELTKNQVSLTCLVKGFYPSDIAVEWESNGQPENNYKTTPPVLDSDGSFALVSKLTVDKSRWQQGNVFSCSVMHEALHNHYTQKSLSLSPG

SEQ ID NO: 96 - DNA, 318 bp, Artificial Sequence
  Description of Artificial Sequence: Synthetic polynucleotide
gggcagcctagagaaccacaggtgtacgtgtaccctccatctagggacgagctgaccaagaaccaggtcagtctgacatgtctggtgaaagggttctatcccagcgatatcgcagtggagtgggaatccaatggacagcctgagaacaattacaagaccacaccccctgtgctggactctgatggaagtttcgccctggtgagtaagctgaccgtcgataaatcacggtggcagcagggcaacgtgttcagctgttcagtgatgcacgaagcactgcacaaccactacacccagaaaagcctgtccctgtcccccggc

SEQ ID NO: 97 - protein, 448 aa, Artificial Sequence
  Description of Artificial Sequence: Synthetic polypeptide
EVQLVESGGGLVQPGGSLRLSCAASGFTFADYTMDWVRQAPGKGLEWVGDVNPNSGGSIYNQRFKGRFTFSVDRSKNTLYLQMNSLRAEDTAVYYCARNLGPSFYFDYWGQGTLVTVSSASTKGPSVFPLAPSSKSTSGGTAALGCLVKDYFPEPVTVSWNSGALTSGVHTFPAVLQSSGLYSLSSVVTVPSSSLGTQTYICNVNHKPSNTKVDKKVEPKSCDKTHTCPPCPAPELLGGPSVFLFPPKPKDTLMISRTPEVTCVVVDVSHEDPEVKFNWYVDGVEVHNAKTKPREEQYNSTYRVVSVLTVLHQDWLNGKEYKCKVSNKALPAPIEKTISKAKGQPREPQVYVYPPSRDELTKNQVSLTCLVKGFYPSDIAVEWESNGQPENNYKTTPPVLDSDGSFALVSKLTVDKSRWQQGNVFSCSVMHEALHNHYTQKSLSLSPG

SEQ ID NO: 98 - DNA, 1344 bp, Artificial Sequence
  Description of Artificial Sequence: Synthetic polynucleotide
gaggtgcagctggtggaatcaggagggggcctggtgcagcccggagggtctctgcgactgtcatgtgccgcttctgggttcactttcgcagactacacaatggattgggtgcgacaggcccccggaaagggactggagtgggtgggcgatgtcaaccctaattctggcgggagtatctacaaccagcggttcaaggggagattcactttttcagtggacagaagcaaaaacaccctgtatctgcagatgaacagcctgagggccgaagataccgctgtctactattgcgctcgcaatctgggccccagtttctactttgactattgggggcagggaaccctggtgacagtcagctccgctagcactaaggggccttccgtgtttccactggctccctctagtaaatccacctctggaggcacagctgcactgggatgtctggtgaaggattacttccctgaaccagtcacagtgagttggaactcaggggctctgacaagtggagtccatacttttcccgcagtgctgcagtcaagcggactgtactccctgtcctctgtggtcaccgtgcctagttcaagcctgggcacccagacatatatctgcaacgtgaatcacaagccatcaaatacaaaagtcgacaagaaagtggagcccaagagctgtgataaaactcatacctgcccaccttgtccggcgccagaactgctgggaggaccaagcgtgttcctgtttccacccaagcctaaagacaccctgatgatttcccggactcctgaggtcacctgcgtggtcgtggacgtgtctcacgaggaccccgaagtcaagttcaactggtacgtggatggcgtcgaagtgcataatgccaagaccaaaccccgggaggaacagtacaactctacctatagagtcgtgagtgtcctgacagtgctgcaccaggactggctgaatgggaaggagtataagtgtaaagtgagcaacaaagccctgcccgccccaatcgaaaaaacaatctctaaagcaaaaggacagcctcgcgaaccacaggtctacgtctaccccccatcaagagatgaactgacaaaaaatcaggtctctctgacatgcctggtcaaaggattctacccttccgacatcgccgtggagtgggaaagtaacggccagcccgagaacaattacaagaccacaccccctgtcctggactctgatgggagtttcgctctggtgtcaaagctgaccgtcgataaaagccggtggcagcagggcaatgtgtttagctgctccgtcatgcacgaagccctgcacaatcactacacacagaagtccctgagcctgagccctggc

SEQ ID NO: 99 - protein, 119 aa, Artificial Sequence
  Description of Artificial Sequence: Synthetic polypeptide
EVQLVESGGGLVQPGGSLRLSCAASGFTFADYTMDWVRQAPGKGLEWVGDVNPNSGGSIYNQRFKGRFTFSVDRSKNTLYLQMNSLRAEDTAVYYCARNLGPSFYFDYWGQGTLVTVSS

SEQ ID NO: 100 - DNA, 357 bp, Artificial Sequence
  Description of Artificial Sequence: Synthetic polynucleotide
gaggtgcagctggtggaatcaggagggggcctggtgcagcccggagggtctctgcgactgtcatgtgccgcttctgggttcactttcgcagactacacaatggattgggtgcgacaggcccccggaaagggactggagtgggtgggcgatgtcaaccctaattctggcgggagtatctacaaccagcggttcaaggggagattcactttttcagtggacagaagcaaaaacaccctgtatctgcagatgaacagcctgagggccgaagataccgctgtctactattgcgctcgcaatctgggccccagtttctactttgactattgggggcagggaaccctggtgacagtcagctcc

SEQ ID NO: 101 - protein, 8 aa, Artificial Sequence
  Description of Artificial Sequence: Synthetic peptide
GFTFADYT

SEQ ID NO: 102 - DNA, 24 bp, Artificial Sequence
  Description of Artificial Sequence: Synthetic oligonucleotide
gggttcactttcgcagactacaca

SEQ ID NO: 103 - protein, 12 aa, Artificial Sequence
  Description of Artificial Sequence: Synthetic peptide
ARNLGPSFYFDY

SEQ ID NO: 104 - DNA, 36 bp, Artificial Sequence
  Description of Artificial Sequence: Synthetic oligonucleotide
gctcgcaatctgggccccagtttctactttgactat

SEQ ID NO: 105 - protein, 8 aa, Artificial Sequence
  Description of Artificial Sequence: Synthetic peptide
VNPNSGGS

SEQ ID NO: 106 - DNA, 24 bp, Artificial Sequence
  Description of Artificial Sequence: Synthetic oligonucleotide
gtcaaccctaattctggcgggagt

SEQ ID NO: 107 - protein, 98 aa, Artificial Sequence; identical to SEQ ID NO: 11
  Description of Artificial Sequence: Synthetic polypeptide

SEQ ID NO: 108 - DNA, 294 bp, Artificial Sequence
  Description of Artificial Sequence: Synthetic polynucleotide
gctagcactaaggggccttccgtgtttccactggctccctctagtaaatccacctctggaggcacagctgcactgggatgtctggtgaaggattacttccctgaaccagtcacagtgagttggaactcaggggctctgacaagtggagtccatacttttcccgcagtgctgcagtcaagcggactgtactccctgtcctctgtggtcaccgtgcctagttcaagcctgggcacccagacatatatctgcaacgtgaatcacaagccatcaaatacaaaagtcgacaagaaagtg

SEQ ID NO: 109 - protein, 110 aa, Artificial Sequence; identical to SEQ ID NO: 13
  Description of Artificial Sequence: Synthetic polypeptide

SEQ ID NO: 110 - DNA, 330 bp, Artificial Sequence
  Description of Artificial Sequence: Synthetic polynucleotide
gcgccagaactgctgggaggaccaagcgtgttcctgtttccacccaagcctaaagacaccctgatgatttcccggactcctgaggtcacctgcgtggtcgtggacgtgtctcacgaggaccccgaagtcaagttcaactggtacgtggatggcgtcgaagtgcataatgccaagaccaaaccccgggaggaacagtacaactctacctatagagtcgtgagtgtcctgacagtgctgcaccaggactggctgaatgggaaggagtataagtgtaaagtgagcaacaaagccctgcccgccccaatcgaaaaaacaatctctaaagcaaaa

SEQ ID NO: 111 - protein, 106 aa, Artificial Sequence; identical to SEQ ID NO: 95
  Description of Artificial Sequence: Synthetic polypeptide

SEQ ID NO: 112 - DNA, 318 bp, Artificial Sequence
  Description of Artificial Sequence: Synthetic polynucleotide
ggacagcctcgcgaaccacaggtctacgtctaccccccatcaagagatgaactgacaaaaaatcaggtctctctgacatgcctggtcaaaggattctacccttccgacatcgccgtggagtgggaaagtaacggccagcccgagaacaattacaagaccacaccccctgtcctggactctgatgggagtttcgctctggtgtcaaagctgaccgtcgataaaagccggtggcagcagggcaatgtgtttagctgctccgtcatgcacgaagccctgcacaatcactacacacagaagtccctgagcctgagccctggc

SEQ ID NO: 113 - protein, 226 aa, Artificial Sequence
  Description of Artificial Sequence: Synthetic polypeptide
YPYDVPDYATGSDIQMTQSPSSLSASVGDRVTITCKASQDVSIGVAWYQQKPGKAPKLLIYSASYRYTGVPSRFSGSGSGTDFTLTISSLQPEDFATYYCQQYYIYPYTFGQGTKVEIKRTVAAPSVFIFPPSDEELKSGTASVVCLLNNFYPREAKVQWKVDNALQSGNSEESVTEQDSKDSTYSLSSTLELSKADYEKHKVYACEVTHQGLSSPVTKSFNRGEC

SEQ ID NO: 114 - DNA, 678 bp, Artificial Sequence
  Description of Artificial Sequence: Synthetic polynucleotide
tatccctacgatgtgcctgactacgctactggctccgatatccagatgacccagtctccaagctccctgagtgcatcagtgggggaccgagtcaccatcacatgcaaggcttcccaggatgtgtctattggagtcgcatggtaccagcagaagccaggcaaagcacccaagctgctgatctacagcgcctcctaccggtatactggggtgccttccagattctctggcagtgggtcaggaaccgactttactctgaccatctctagtctgcagcccgaggatttcgccacctactattgccagcagtactatatctacccttatacctttggccaggggacaaaagtggagatcaagaggacagtggccgctccaagtgtcttcatttttcccccttccgacgaagagctgaaaagtggaactgcttcagtggtctgtctgctgaacaatttctacccccgcgaagccaaagtgcagtggaaggtcgataacgctctgcagagcggcaattccgaggagtctgtgacagaacaggacagtaaagattcaacttatagcctgtcaagcacactggagctgtctaaggcagactacgagaagcacaaagtgtatgcctgcgaagtcacccatcaggggctgtcctctcccgtgacaaagagctttaacagaggagagtgt

SEQ ID NO: 115 - protein, 107 aa, Artificial Sequence [sequence omitted]

SEQ ID NO: 116 - DNA, 321 bp, Artificial Sequence
  Description of Artificial Sequence: Synthetic polynucleotide
gatatccagatgacccagtctccaagctccctgagtgcatcagtgggggaccgagtcaccatcacatgcaaggcttcccaggatgtgtctattggagtcgcatggtaccagcagaagccaggcaaagcacccaagctgctgatctacagcgcctcctaccggtatactggggtgccttccagattctctggcagtgggtcaggaaccgactttactctgaccatctctagtctgcagcccgaggatttcgccacctactattgccagcagtactatatctacccttatacctttggccaggggacaaaagtggagatcaag

SEQ ID NO: 117 - protein, 6 aa, Artificial Sequence
  Description of Artificial Sequence: Synthetic peptide
QDVSIG

SEQ ID NO: 118 - DNA, 18 bp, Artificial Sequence
  Description of Artificial Sequence: Synthetic oligonucleotide
caggatgtgtctattgga

SEQ ID NO: 119 - protein, 9 aa, Artificial Sequence
  Description of Artificial Sequence: Synthetic peptide
QQYYIYPYT

SEQ ID NO: 120 - DNA, 27 bp, Artificial Sequence
  Description of Artificial Sequence: Synthetic oligonucleotide
cagcagtactatatctacccttatacc

SEQ ID NO: 121 - protein, 3 aa, Artificial Sequence
  Description of Artificial Sequence: Synthetic peptide
SAS

SEQ ID NO: 122 - DNA, 9 bp, Artificial Sequence
  Description of Artificial Sequence: Synthetic oligonucleotide
agcgcctcc

SEQ ID NO: 123 - protein, 107 aa, Artificial Sequence
  Description of Artificial Sequence: Synthetic polypeptide
RTVAAPSVFIFPPSDEELKSGTASVVCLLNNFYPREAKVQWKVDNALQSGNSEESVTEQDSKDSTYSLSSTLELSKADYEKHKVYACEVTHQGLSSPVTKSFNRGEC

SEQ ID NO: 124 - DNA, 321 bp, Artificial Sequence
  Description of Artificial Sequence: Synthetic polynucleotide
aggacagtggccgctccaagtgtcttcatttttcccccttccgacgaagagctgaaaagtggaactgcttcagtggtctgtctgctgaacaatttctacccccgcgaagccaaagtgcagtggaaggtcgataacgctctgcagagcggcaattccgaggagtctgtgacagaacaggacagtaaagattcaacttatagcctgtcaagcacactggagctgtctaaggcagactacgagaagcacaaagtgtatgcctgcgaagtcacccatcaggggctgtcctctcccgtgacaaagagctttaacagaggagagtgt

SEQ ID NO: 125 - protein, 450 aa, Artificial Sequence
  Description of Artificial Sequence: Synthetic polypeptide
EVQLVESGGGLVQPGGSLRLSCAASGFNIKDTYIHWVRQAPGKGLEWVARIYPTNGYTRYADSVKGRFTISADTSKNTAYLQMNSLRAEDTAVYYCSRWGGDGFYAMDYWGQGTLVTVSSASTKGPSVFPLAPSSKSTSGGTAALGCLVKDYFPEPVTVSWNSGALTSGVHTFPAVLQSSGLYSLSSVVTVPSSSLGTQTYICNVNHKPSNTKVDKKVEPKSCDKTHTCPPCPAPELLGGPSVFLFPPKPKDTLMISRTPEVTCVVVDVSHEDPEVKFNWYVDGVEVHNAKTKPREEQYNSTYRVVSVLTVLHQDWLNGKEYKCKVSNKALPAPIEKTISKAKGQPREPQVYVYPPSRDELTKNQVSLTCLVKGFYPSDIAVEWESNGQPENNYKTTPPVLDSDGSFALVSKLTVDKSRWQQGNVFSCSVMHEALHNHYTQKSLSLSPGK

SEQ ID NO: 126 - DNA, 1350 bp, Artificial Sequence
  Description of Artificial Sequence: Synthetic polynucleotide
gaagtccagctggtcgaaagcggaggaggactggtgcagccaggagggtctctgcgactgagttgcgccgcttcaggcttcaacatcaaggacacctacattcactgggtgcgccaggctcctggaaaaggcctggagtgggtggcacgaatctatccaactaatggatacacccggtatgcagacagcgtgaagggccggttcaccattagcgcagatacatccaaaaacactgcctacctgcagatgaacagcctgcgagccgaagatactgctgtgtactattgcagtcggtggggaggcgacggcttctacgctatggattattgggggcagggaaccctggtcacagtgagctccgcatctacaaaggggcctagtgtgtttccactggccccctctagtaaatccacctctgggggaacagcagccctgggatgtctggtgaaggactatttcccagagcccgtcactgtgagttggaactcaggcgccctgacatccggggtccatacttttcctgctgtgctgcagtcaagcggcctgtactctctgtcctctgtggtcaccgtgccaagttcaagcctggggactcagacctatatctgcaacgtgaatcacaagccaagcaatacaaaagtcgacaagaaagtggaacccaagagctgtgataaaacacatacttgccccccttgtcctgcaccagagctgctgggaggaccatccgtgttcctgtttccacccaagcctaaagacaccctgatgatttccaggactccagaagtcacctgcgtggtcgtggacgtgtctcacgaggaccccgaagtcaagttcaactggtacgtggatggcgtcgaggtgcataatgccaagacaaaacccagggaggaacagtacaactcaacttatcgcgtcgtgagcgtcctgaccgtgctgcaccaggactggctgaacggcaaggagtataagtgcaaagtgagcaataaggctctgcccgcacctatcgagaaaaccattagcaaggccaaagggcagcctagagaaccacaggtctacgtgtatcctccaagcagggacgagctgaccaagaaccaggtctccctgacatgtctggtgaaagggttttaccccagtgatatcgctgtggagtgggaatcaaatggacagcctgaaaacaattataagaccacaccccctgtgctggacagcgatggcagcttcgctctggtctccaagctgactgtggataaatctcggtggcagcagggcaacgtctttagttgttcagtgatgcatgaggcactgcacaatcattacacccagaagagcctgtccctgtctcccggcaaa

SEQ ID NO: 127 - protein, 120 aa, Artificial Sequence [sequence omitted]

SEQ ID NO: 128 - DNA, 360 bp, Artificial Sequence
  Description of Artificial Sequence: Synthetic polynucleotide
gaagtccagctggtcgaaagcggaggaggactggtgcagccaggagggtctctgcgactgagttgcgccgcttcaggcttcaacatcaaggacacctacattcactgggtgcgccaggctcctggaaaaggcctggagtgggtggcacgaatctatccaactaatggatacacccggtatgcagacagcgtgaagggccggttcaccattagcgcagatacatccaaaaacactgcctacctgcagatgaacagcctgcgagccgaagatactgctgtgtactattgcagtcggtggggaggcgacggcttctacgctatggattattgggggcagggaaccctggtcacagtgagctcc

SEQ ID NO: 129 - protein, 8 aa, Artificial Sequence
  Description of Artificial Sequence: Synthetic peptide
GFNIKDTY

SEQ ID NO: 130 - DNA, 24 bp, Artificial Sequence
  Description of Artificial Sequence: Synthetic oligonucleotide
ggcttcaacatcaaggacacctac

SEQ ID NO: 131 - protein, 13 aa, Artificial Sequence
  Description of Artificial Sequence: Synthetic peptide
SRWGGDGFYAMDY

SEQ ID NO: 132 - DNA, 39 bp, Artificial Sequence
  Description of Artificial Sequence: Synthetic oligonucleotide
agtcggtggggaggcgacggcttctacgctatggattat

SEQ ID NO: 133 - protein, 8 aa, Artificial Sequence
  Description of Artificial Sequence: Synthetic peptide
IYPTNGYT

SEQ ID NO: 134 - DNA, 24 bp, Artificial Sequence
  Description of Artificial Sequence: Synthetic oligonucleotide
atctatccaactaatggatacacc

SEQ ID NO: 135 - protein, 98 aa, Artificial Sequence; identical to SEQ ID NO: 11
  Description of Artificial Sequence: Synthetic polypeptide

SEQ ID NO: 136 - DNA, 294 bp, Artificial Sequence
  Description of Artificial Sequence: Synthetic polynucleotide
gcatctacaaaggggcctagtgtgtttccactggccccctctagtaaatccacctctgggggaacagcagccctgggatgtctggtgaaggactatttcccagagcccgtcactgtgagttggaactcaggcgccctgacatccggggtccatacttttcctgctgtgctgcagtcaagcggcctgtactctctgtcctctgtggtcaccgtgccaagttcaagcctggggactcagacctatatctgcaacgtgaatcacaagccaagcaatacaaaagtcgacaagaaagtg

SEQ ID NO: 137 - protein, 110 aa, Artificial Sequence; identical to SEQ ID NO: 13
  Description of Artificial Sequence: Synthetic polypeptide

SEQ ID NO: 138 - DNA, 330 bp, Artificial Sequence
  Description of Artificial Sequence: Synthetic polynucleotide
gcaccagagctgctgggaggaccatccgtgttcctgtttccacccaagcctaaagacaccctgatgatttccaggactccagaagtcacctgcgtggtcgtggacgtgtctcacgaggaccccgaagtcaagttcaactggtacgtggatggcgtcgaggtgcataatgccaagacaaaacccagggaggaacagtacaactcaacttatcgcgtcgtgagcgtcctgaccgtgctgcaccaggactggctgaacggcaaggagtataagtgcaaagtgagcaataaggctctgcccgcacctatcgagaaaaccattagcaaggccaaa

SEQ ID NO: 139 - protein, 106 aa, Artificial Sequence; identical to SEQ ID NO: 95
  Description of Artificial Sequence: Synthetic polypeptide

SEQ ID NO: 140 - DNA, 318 bp, Artificial Sequence
  Description of Artificial Sequence: Synthetic polynucleotide
gggcagcctagagaaccacaggtctacgtgtatcctccaagcagggacgagctgaccaagaaccaggtctccctgacatgtctggtgaaagggttttaccccagtgatatcgctgtggagtgggaatcaaatggacagcctgaaaacaattataagaccacaccccctgtgctggacagcgatggcagcttcgctctggtctccaagctgactgtggataaatctcggtggcagcagggcaacgtctttagttgttcagtgatgcatgaggcactgcacaatcattacacccagaagagcctgtccctgtctcccggc

SEQ ID NO: 141 - protein, 232 aa, Artificial Sequence
  Description of Artificial Sequence: Synthetic polypeptide
EPKSSDKTHTCPPCPAPELLGGPSVFLFPPKPKDTLMISRTPEVTCVVVDVSHEDPEVKFNWYVDGVEVHNAKTKPREEQYNSTYRVVSVLTVLHQDWLNGKEYKCKVSNKALPAPIEKTISKAKGQPREPQVYTLPPSRDELTKNQVSLICLVKGFYPSDIAVEWESNGQPENRYMTWPPVLDSDGSFFLYSKLTVDKSRWQQGNVFSCSVMHEALHNHYTQKSLSLSPGK

SEQ ID NO: 142 - DNA, 696 bp, Artificial Sequence
  Description of Artificial Sequence: Synthetic polynucleotide
gagcccaagagcagcgataagacccacacctgccctccctgtccagctccagaactgctgggaggacctagcgtgttcctgtttccccctaagccaaaagacactctgatgatttccaggactcccgaggtgacctgcgtggtggtggacgtgtctcacgaggaccccgaagtgaagttcaactggtacgtggatggcgtggaagtgcataatgctaagacaaaaccaagagaggaacagtacaactccacttatcgcgtcgtgagcgtgctgaccgtgctgcaccaggactggctgaacgggaaggagtataagtgcaaagtcagtaataaggccctgcctgctccaatcgaaaaaaccatctctaaggccaaaggccagccaagggagccccaggtgtacacactgccacccagcagagacgaactgaccaagaaccaggtgtccctgatctgtctggtgaaaggcttctatcctagtgatattgctgtggagtgggaatcaaatggacagccagagaacagatacatgacctggcctccagtgctggacagcgatggcagcttcttcctgtattccaagctgacagtggataaatctcgatggcagcaggggaacgtgtttagttgttcagtgatgcatgaagccctgcacaatcattacactcagaagagcctgtccctgtctcccggcaaa

SEQ ID NO: 143 - protein, 110 aa, Artificial Sequence; identical to SEQ ID NO: 13
  Description of Artificial Sequence: Synthetic polypeptide

SEQ ID NO: 144 - DNA, 330 bp, Artificial Sequence; identical to SEQ ID NO: 14
  Description of Artificial Sequence: Synthetic polynucleotide

SEQ ID NO: 145 - protein, 106 aa, Artificial Sequence
  Description of Artificial Sequence: Synthetic polypeptide
GQPREPQVYTLPPSRDELTKNQVSLICLVKGFYPSDIAVEWESNGQPENRYMTWPPVLDSDGSFFLYSKLTVDKSRWQQGNVFSCSVMHEALHNHYTQKSLSLSPG

SEQ ID NO: 146 - DNA, 318 bp, Artificial Sequence
  Description of Artificial Sequence: Synthetic polynucleotide
ggccagccaagggagccccaggtgtacacactgccacccagcagagacgaactgaccaagaaccaggtgtccctgatctgtctggtgaaaggcttctatcctagtgatattgctgtggagtgggaatcaaatggacagccagagaacagatacatgacctggcctccagtgctggacagcgatggcagcttcttcctgtattccaagctgacagtggataaatctcgatggcagcaggggaacgtgtttagttgttcagtgatgcatgaagccctgcacaatcattacactcagaagagcctgtccctgtctcccggc

SEQ ID NO: 147 - protein, 481 aa, Artificial Sequence
  Description of Artificial Sequence: Synthetic polypeptide
DIQMTQSPSSLSASVGDRVTITCRASQDVNTAVAWYQQKPGKAPKLLIYSASFLYSGVPSRFSGSRSGTDFTLTISSLQPEDFATYYCQQHYTTPPTFGQGTKVEIKGGSGGGSGGGSGGGSGGGSGEVQLVESGGGLVQPGGSLRLSCAASGFNIKDTYIHWVRQAPGKGLEWVARIYPTNGYTRYADSVKGRFTISADTSKNTAYLQMNSLRAEDTAVYYCSRWGGDGFYAMDYWGQGTLVTVSSAAEPKSSDKTHTCPPCPAPELLGGPSVFLFPPKPKDTLMISRTPEVTCVVVDVSHEDPEVKFNWYVDGVEVHNAKTKPREEQYNSTYRVVSVLTVLHQDWLNGKEYKCKVSNKALPAPIEKTISKAKGQPREPQVYTYPPSRDELTKNQVSLTCLVKGFYPSDIAVEWESNGQPENNYKTTPPVLDEDGSFALVSKLTVDKSRWQQGNVFSCSVMHEALHNHYTQKSLSLSPGK

SEQ ID NO: 148 - DNA, 1443 bp, Artificial Sequence
  Description of Artificial Sequence: Synthetic polynucleotide
gacatccagatgacccagtctccatcctccctgtctgcatctgtaggagacagagtcaccatcacttgccgggcaagtcaggacgttaacaccgctgtagcttggtatcagcagaaaccagggaaagcccctaagctcctgatctattctgcatcctttttgtacagtggggtcccatcaaggttcagtggcagtcgatctgggacagatttcactctcaccatcagcagtctgcaacctgaagattttgcaacttactactgtcaacagcattacactaccccacccactttcggccaagggaccaaagtggagatcaaaggtggttctggtggtggttctggtggtggttctggtggtggttctggtggtggttctggtgaagtgcagctggtggagtctgggggaggcttggtacagcctggcgggtccctgagactctcctgtgcagcctctggattcaacattaaagatacttatatccactgggtccggcaagctccagggaagggcctggagtgggtcgcacgtatttatcccacaaatggttacacacggtatgcggactctgtgaagggccgattcaccatctccgcagacacttccaagaacaccgcgtatctgcaaatgaacagtctgagagctgaggacacggccgtttattactgttcaagatggggcggagacggtttctacgctatggactactggggccaagggaccctggtcaccgtctcctcagccgccgagcccaagagcagcgataagacccacacctgccctccctgtccagctccagaactgctgggaggacctagcgtgttcctgtttccccctaagccaaaagacactctgatgatttccaggactcccgaggtgacctgcgtggtggtggacgtgtctcacgaggaccccgaagtgaagttcaactggtacgtggatggcgtggaagtgcataatgctaagacaaaaccaagagaggaacagtacaactccacttatcgcgtcgtgagcgtgctgaccgtgctgcaccaggactggctgaacgggaaggagtataagtgcaaagtcagtaataaggccctgcctgctccaatcgaaaaaaccatctctaaggccaaaggccagccaagggagccccaggtgtacacatacccacccagcagagacgaactgaccaagaaccaggtgtccctgacatgtctggtgaaaggcttctatcctagtgatattgctgtggagtgggaatcaaatggacagccagagaacaattacaagaccacacctccagtgctggacgaggatggcagcttcgccctggtgtccaagctgacagtggataaatctcgatggcagcaggggaacgtgtttagttgttcagtgatgcatgaagccctgcacaatcattacactcagaagagcctgtccctgtctcccggcaaa

SEQ ID NO: 149 - protein, 107 aa, Artificial Sequence [sequence omitted]

SEQ ID NO: 150 - DNA, 321 bp, Artificial Sequence
  Description of Artificial Sequence: Synthetic polynucleotide
gacatccagatgacccagtctccatcctccctgtctgcatctgtaggagacagagtcaccatcacttgccgggcaagtcaggacgttaacaccgctgtagcttggtatcagcagaaaccagggaaagcccctaagctcctgatctattctgcatcctttttgtacagtggggtcccatcaaggttcagtggcagtcgatctgggacagatttcactctcaccatcagcagtctgcaacctgaagattttgcaacttactactgtcaacagcattacactaccccacccactttcggccaagggaccaaagtggagatcaaa

SEQ ID NO: 151 - protein, 6 aa, Artificial Sequence
  Description of Artificial Sequence: Synthetic peptide
QDVNTA

SEQ ID NO: 152 - DNA, 18 bp, Artificial Sequence
  Description of Artificial Sequence: Synthetic oligonucleotide
caggacgttaacaccgct

SEQ ID NO: 153 - protein, 9 aa, Artificial Sequence
  Description of Artificial Sequence: Synthetic peptide
QQHYTTPPT

SEQ ID NO: 154 - DNA, 27 bp, Artificial Sequence
  Description of Artificial Sequence: Synthetic oligonucleotide
caacagcattacactaccccacccact

SEQ ID NO: 155 - protein, 3 aa, Artificial Sequence
  Description of Artificial Sequence: Synthetic peptide
SAS

SEQ ID NO: 156 - DNA, 9 bp, Artificial Sequence
  Description of Artificial Sequence: Synthetic oligonucleotide
tctgcatcc

SEQ ID NO: 157 - protein, 120 aa, Artificial Sequence [sequence omitted]

SEQ ID NO: 158 - DNA, 360 bp, Artificial Sequence
  Description of Artificial Sequence: Synthetic polynucleotide
gaagtgcagctggtggagtctgggggaggcttggtacagcctggcgggtccctgagactctcctgtgcagcctctggattcaacattaaagatacttatatccactgggtccggcaagctccagggaagggcctggagtgggtcgcacgtatttatcccacaaatggttacacacggtatgcggactctgtgaagggccgattcaccatctccgcagacacttccaagaacaccgcgtatctgcaaatgaacagtctgagagctgaggacacggccgtttattactgttcaagatggggcggagacggtttctacgctatggactactggggccaagggaccctggtcaccgtctcctca

SEQ ID NO: 159 - protein, 8 aa, Artificial Sequence
  Description of Artificial Sequence: Synthetic peptide
GFNIKDTY

SEQ ID NO: 160 - DNA, 24 bp, Artificial Sequence
  Description of Artificial Sequence: Synthetic oligonucleotide
ggattcaacattaaagatacttat

SEQ ID NO: 161 - protein, 13 aa, Artificial Sequence
  Description of Artificial Sequence: Synthetic peptide
SRWGGDGFYAMDY

SEQ ID NO: 162 - DNA, 39 bp, Artificial Sequence
  Description of Artificial Sequence: Synthetic oligonucleotide
tcaagatggggcggagacggtttctacgctatggactac

SEQ ID NO: 163 - protein, 8 aa, Artificial Sequence
  Description of Artificial Sequence: Synthetic peptide
IYPTNGYT

SEQ ID NO: 164 - DNA, 24 bp, Artificial Sequence
  Description of Artificial Sequence: Synthetic oligonucleotide
atttatcccacaaatggttacaca

SEQ ID NO: 165 - protein, 110 aa, Artificial Sequence; identical to SEQ ID NO: 13
  Description of Artificial Sequence: Synthetic polypeptide

SEQ ID NO: 166 - DNA, 330 bp, Artificial Sequence; identical to SEQ ID NO: 14
  Description of Artificial Sequence: Synthetic polynucleotide

SEQ ID NO: 167 - protein, 106 aa, Artificial Sequence
  Description of Artificial Sequence: Synthetic polypeptide
GQPREPQVYTYPPSRDELTKNQVSLTCLVKGFYPSDIAVEWESNGQPENNYKTTPPVLDEDGSFALVSKLTVDKSRWQQGNVFSCSVMHEALHNHYTQKSLSLSPG

SEQ ID NO: 168 - DNA, 318 bp, Artificial Sequence
  Description of Artificial Sequence: Synthetic polynucleotide
ggccagccaagggagccccaggtgtacacatacccacccagcagagacgaactgaccaagaaccaggtgtccctgacatgtctggtgaaaggcttctatcctagtgatattgctgtggagtgggaatcaaatggacagccagagaacaattacaagaccacacctccagtgctggacgaggatggcagcttcgccctggtgtccaagctgacagtggataaatctcgatggcagcaggggaacgtgtttagttgttcagtgatgcatgaagccctgcacaatcattacactcagaagagcctgtccctgtctcccggc

SEQ ID NO: 169 - protein, 481 aa, Artificial Sequence
  Description of Artificial Sequence: Synthetic polypeptide
DIQMTQSPSSLSASVGDRVTITCRASQDVNTAVAWYQQKPGKAPKLLIYSASFLYSGVPSRFSGSRSGTDFTLTISSLQPEDFATYYCQQHYTTPPTFGQGTKVEIKGGSGGGSGGGSGGGSGGGSGEVQLVESGGGLVQPGGSLRLSCAASGFNIKDTYIHWVRQAPGKGLEWVARIYPTNGYTRYADSVKGRFTISADTSKNTAYLQMNSLRAEDTAVYYCSRWGGDGFYAMDYWGQGTLVTVSSAAEPKSSDKTHTCPPCPAPELLGGPSVFLFPPKPKDTLMISRTPEVTCVVVDVSHEDPEVKFNWYVDGVEVHNAKTKPREEQYNSTYRVVSVLTVLHQDWLNGKEYKCKVSNKALPAPIEKTISKAKGQPREPQVYTLPPSRDELTKNQVSLICLVKGFYPSDIAVEWESNGQPENRYMTWPPVLDSDGSFFLYSKLTVDKSRWQQGNVFSCSVMHEALHNHYTQKSLSLSPGK

SEQ ID NO: 170 - DNA, 1443 bp, Artificial Sequence
  Description of Artificial Sequence: Synthetic polynucleotide
gacatccagatgacccagtctccatcctccctgtctgcatctgtaggagacagagtcaccatcacttgccgggcaagtcaggacgttaacaccgctgtagcttggtatcagcagaaaccagggaaagcccctaagctcctgatctattctgcatcctttttgtacagtggggtcccatcaaggttcagtggcagtcgatctgggacagatttcactctcaccatcagcagtctgcaacctgaagattttgcaacttactactgtcaacagcattacactaccccacccactttcggccaagggaccaaagtggagatcaaaggtggttctggtggtggttctggtggtggttctggtggtggttctggtggtggttctggtgaagtgcagctggtggagtctgggggaggcttggtacagcctggcgggtccctgagactctcctgtgcagcctctggattcaacattaaagatacttatatccactgggtccggcaagctccagggaagggcctggagtgggtcgcacgtatttatcccacaaatggttacacacggtatgcggactctgtgaagggccgattcaccatctccgcagacacttccaagaacaccgcgtatctgcaaatgaacagtctgagagctgaggacacggccgtttattactgttcaagatggggcggagacggtttctacgctatggactactggggccaagggaccctggtcaccgtctcctcagccgccgagcccaagagcagcgataagacccacacctgccctccctgtccagctccagaactgctgggaggacctagcgtgttcctgtttccccctaagccaaaagacactctgatgatttccaggactcccgaggtgacctgcgtggtggtggacgtgtctcacgaggaccccgaagtgaagttcaactggtacgtggatggcgtggaagtgcataatgctaagacaaaaccaagagaggaacagtacaactccacttatcgcgtcgtgagcgtgctgaccgtgctgcaccaggactggctgaacgggaaggagtataagtgcaaagtcagtaataaggccctgcctgctccaatcgaaaaaaccatctctaaggccaaaggccagccaagggagccccaggtgtacacactgccacccagcagagacgaactgaccaagaaccaggtgtccctgatctgtctggtgaaaggcttctatcctagtgatattgctgtggagtgggaatcaaatggacagccagagaacagatacatgacctggcctccagtgctggacagcgatggcagcttcttcctgtattccaagctgacagtggataaatctcgatggcagcaggggaacgtgtttagttgttcagtgatgcatgaagccctgcacaatcattacactcagaagagcctgtccctgtctcccggcaaa

SEQ ID NO: 171 - protein, 107 aa, Artificial Sequence [sequence omitted]

SEQ ID NO: 172 - DNA, 321 bp, Artificial Sequence; identical to SEQ ID NO: 150
  Description of Artificial Sequence: Synthetic polynucleotide

SEQ ID NO: 173 - protein, 6 aa, Artificial Sequence
  Description of Artificial Sequence: Synthetic peptide
QDVNTA

SEQ ID NO: 174 - DNA, 18 bp, Artificial Sequence
  Description of Artificial Sequence: Synthetic oligonucleotide
caggacgttaacaccgct

SEQ ID NO: 175 - protein, 9 aa, Artificial Sequence
  Description of Artificial Sequence: Synthetic peptide
QQHYTTPPT

SEQ ID NO: 176 - DNA, 27 bp, Artificial Sequence
  Description of Artificial Sequence: Synthetic oligonucleotide
caacagcattacactaccccacccact

SEQ ID NO: 177 - protein, 3 aa, Artificial Sequence
  Description of Artificial Sequence: Synthetic peptide
SAS

SEQ ID NO: 178 - DNA, 9 bp, Artificial Sequence
  Description of Artificial Sequence: Synthetic oligonucleotide
tctgcatcc

SEQ ID NO: 179 - protein, 120 aa, Artificial Sequence [sequence omitted]

SEQ ID NO: 180 - DNA, 360 bp, Artificial Sequence; identical to SEQ ID NO: 158
  Description of Artificial Sequence: Synthetic polynucleotide

SEQ ID NO: 181 - protein, 8 aa, Artificial Sequence
  Description of Artificial Sequence: Synthetic peptide
GFNIKDTY

SEQ ID NO: 182 - DNA, 24 bp, Artificial Sequence
  Description of Artificial Sequence: Synthetic oligonucleotide
ggattcaacattaaagatacttat

SEQ ID NO: 183 - protein, 13 aa, Artificial Sequence
  Description of Artificial Sequence: Synthetic peptide
SRWGGDGFYAMDY

SEQ ID NO: 184 - DNA, 39 bp, Artificial Sequence; identical to SEQ ID NO: 162
  Description of Artificial Sequence: Synthetic oligonucleotide

SEQ ID NO: 185 - protein, 8 aa, Artificial Sequence
  Description of Artificial Sequence: Synthetic peptide
IYPTNGYT

SEQ ID NO: 186 - DNA, 24 bp, Artificial Sequence
  Description of Artificial Sequence: Synthetic oligonucleotide
atttatcccacaaatggttacaca

SEQ ID NO: 187 - protein, 110 aa, Artificial Sequence; identical to SEQ ID NO: 13
  Description of Artificial Sequence: Synthetic polypeptide

SEQ ID NO: 188 - DNA, 330 bp, Artificial Sequence; identical to SEQ ID NO: 14
  Description of Artificial Sequence: Synthetic polynucleotide

SEQ ID NO: 189 - protein, 106 aa, Artificial Sequence; identical to SEQ ID NO: 145
  Description of Artificial Sequence: Synthetic polypeptide

SEQ ID NO: 190 - DNA, 318 bp, Artificial Sequence; identical to SEQ ID NO: 146
  Description of Artificial Sequence: Synthetic polynucleotide

SEQ ID NO: 191 - protein, 214 aa, Artificial Sequence
  Description of Artificial Sequence: Synthetic polypeptide
DIQMTQSPSSLSASVGDRVTITCRASQDVNTAVAWYQQKPGKAPKLLIYSASFLYSGVPSRFSGSRSGTDFTLTISSLQPEDFATYYCQQHYTTPPTFGQGTKVEIKRTVAAPSVFIFPPSDEQLKSGTASVVCLLNNFYPREAKVQWKVDNALQSGNSQESVTEQDSKDSTYSLSSTLTLSKADYEKHKVYACEVTHQGLSSPVTKSFNRGEC

SEQ ID NO: 192 - DNA, 642 bp, Artificial Sequence
  Description of Artificial Sequence: Synthetic polynucleotide
gatattcagatgacccagtcccctagctccctgtccgcttctgtgggcgacagggtcactatcacctgccgcgcatctcaggatgtgaacaccgcagtcgcctggtaccagcagaagcctgggaaagctccaaagctgctgatctacagtgcatcattcctgtattcaggagtgcccagccggtttagcggcagcagatctggcaccgacttcacactgactatctctagtctgcagcctgaggattttgccacatactattgccagcagcactataccacaccccctactttcggccaggggaccaaagtggagatcaagcgaactgtggccgctccaagtgtcttcatttttccacccagcgacgaacagctgaaatccggcacagcttctgtggtctgtctgctgaacaacttctaccccagagaggccaaagtgcagtggaaggtcgataacgctctgcagagtggcaacagccaggagagcgtgacagaacaggactccaaagattctacttatagtctgtcaagcaccctgacactgagcaaggcagactacgaaaagcataaagtgtatgcctgtgaggtgacccatcaggggctgtcttctcccgtgaccaagtctttcaaccgaggcgaatgt

SEQ ID NO: 193 - protein, 107 aa, Artificial Sequence [sequence omitted]

SEQ ID NO: 194 - DNA, 321 bp, Artificial Sequence
  Description of Artificial Sequence: Synthetic polynucleotide
gatattcagatgacccagtcccctagctccctgtccgcttctgtgggcgacagggtcactatcacctgccgcgcatctcaggatgtgaacaccgcagtcgcctggtaccagcagaagcctgggaaagctccaaagctgctgatctacagtgcatcattcctgtattcaggagtgcccagccggtttagcggcagcagatctggcaccgacttcacactgactatctctagtctgcagcctgaggattttgccacatactattgccagcagcactataccacaccccctactttcggccaggggaccaaagtggagatcaag

SEQ ID NO: 195 - protein, 6 aa, Artificial Sequence
  Description of Artificial Sequence: Synthetic peptide
QDVNTA

SEQ ID NO: 196 - DNA, 18 bp, Artificial Sequence
  Description of Artificial Sequence: Synthetic oligonucleotide
caggatgtgaacaccgca

SEQ ID NO: 197 - protein, 9 aa, Artificial Sequence
  Description of Artificial Sequence: Synthetic peptide
QQHYTTPPT

SEQ ID NO: 198 - DNA, 27 bp, Artificial Sequence
  Description of Artificial Sequence: Synthetic oligonucleotide
cagcagcactataccacaccccctact

SEQ ID NO: 199 - protein, 3 aa, Artificial Sequence
  Description of Artificial Sequence: Synthetic peptide
SAS

SEQ ID NO: 200 - DNA, 9 bp, Artificial Sequence
  Description of Artificial Sequence: Synthetic oligonucleotide
agtgcatca

SEQ ID NO: 201 - protein, 107 aa, Artificial Sequence [sequence omitted]

SEQ ID NO: 202 - DNA, 321 bp, Artificial Sequence
  Description of Artificial Sequence: Synthetic polynucleotide
cgaactgtggccgctccaagtgtcttcatttttccacccagcgacgaacagctgaaatccggcacagcttctgtggtctgtctgctgaacaacttctaccccagagaggccaaagtgcagtggaaggtcgataacgctctgcagagtggcaacagccaggagagcgtgacagaacaggactccaaagattctacttatagtctgtcaagcaccctgacactgagcaaggcagactacgaaaagcataaagtgtatgcctgtgaggtgacccatcaggggctgtcttctcccgtgaccaagtctttcaaccgaggcgaatgt

SEQ ID NO: 203 - protein, 448 aa, Artificial Sequence
  Description of Artificial Sequence: Synthetic polypeptide
EVQLVESGGGLVQPGGSLRLSCAASGFTFTDYTMDWVRQAPGKGLEWVADVNPNSGGSIYNQRFKGRFTLSVDRSKNTLYLQMNSLRAEDTAVYYCARNLGPSFYFDYWGQGTLVTVSSASTKGPSVFPLAPSSKSTSGGTAALGCLVKDYFPEPVTVSWNSGALTSGVHTFPAVLQSSGLYSLSSVVTVPSSSLGTQTYICNVNHKPSNTKVDKKVEPKSCDKTHTCPPCPAPELLGGPSVFLFPPKPKDTLMISRTPEVTCVVVDVSHEDPEVKFNWYVDGVEVHNAKTKPREEQYNSTYRVVSVLTVLHQDWLNGKEYKCKVSNKALPAPIEKTISKAKGQPREPQVYVLPPSRDELTKNQVSLLCLVKGFYPSDIAVEWESNGQPENNYLTWPPVLDSDGSFFLYSKLTVDKSRWQQGNVFSCSVMHEALHNHYTQKSLSLSPG

SEQ ID NO: 204 - DNA, 1344 bp, Artificial Sequence
  Description of Artificial Sequence: Synthetic polynucleotide
gaagtgcagctggtcgaatctggaggaggactggtgcagccaggagggtccctgcgcctgtcttgcgccgctagtggcttcacttttaccgactacaccatggattgggtgcgacaggcacctggaaagggcctggagtgggtcgccgatgtgaacccaaatagcggaggctccatctacaaccagcggttcaagggccggttcaccctgtcagtggaccggagcaaaaacaccctgtatctgcagatgaatagcctgcgagccgaagatactgctgtgtactattgcgcccggaatctggggccctccttctactttgactattgggggcagggaactctggtcaccgtgagctccgcctccaccaagggaccttctgtgttcccactggctccctctagtaaatccacatctgggggaactgcagccctgggctgtctggtgaaggactacttcccagagcccgtcacagtgtcttggaacagtggcgctctgacttctggggtccacacctttcctgcagtgctgcagtcaagcgggctgtacagcctgtcctctgtggtcaccgtgccaagttcaagcctgggaacacagacttatatctgcaacgtgaatcacaagccatccaatacaaaagtcgacaagaaagtggaacccaagtcttgtgataaaacccatacatgccccccttgtcctgcaccagagctgctgggaggaccaagcgtgttcctgtttccacccaagcctaaagatacactgatgattagtaggaccccagaagtcacatgcgtggtcgtggacgtgagccacgaggaccccgaagtcaagtttaactggtacgtggacggcgtcgaggtgcataatgccaagactaaacccagggaggaacagtacaacagtacctatcgcgtcgtgtcagtcctgacagtgctgcatcaggattggctgaacgggaaagagtataagtgcaaagtgagcaataaggctctgcccgcacctatcgagaaaacaatttccaaggcaaaaggacagcctagagaaccacaggtgtacgtgctgcctccatcaagggatgagctgacaaagaaccaggtcagcctgctgtgtctggtgaaaggattctatccctctgacattgctgtggagtgggaaagtaatggccagcctgagaacaattacctgacctggccccctgtgctggactcagatggcagcttctttctgtatagcaagctgaccgtcgacaaatcccggtggcagcaggggaatgtgtttagttgttcagtcatgcacgaggcactgcacaaccattacacccagaagtcactgtcactgtcaccaggg

SEQ ID NO: 205 - protein, 119 aa, Artificial Sequence [sequence omitted]

SEQ ID NO: 206 - DNA, 357 bp, Artificial Sequence; identical to SEQ ID NO: 20
  Description of Artificial Sequence: Synthetic polynucleotide

SEQ ID NO: 207 - protein, 8 aa, Artificial Sequence
  Description of Artificial Sequence: Synthetic peptide
GFTFTDYT

SEQ ID NO: 208 - DNA, 24 bp, Artificial Sequence
  Description of Artificial Sequence: Synthetic oligonucleotide
ggcttcacttttaccgactacacc

SEQ ID NO: 209 - protein, 12 aa, Artificial Sequence
  Description of Artificial Sequence: Synthetic peptide
ARNLGPSFYFDY

SEQ ID NO: 210 - DNA, 36 bp, Artificial Sequence; identical to SEQ ID NO: 24
  Description of Artificial Sequence: Synthetic oligonucleotide

SEQ ID NO: 211 - protein, 8 aa, Artificial Sequence
  Description of Artificial Sequence: Synthetic peptide
VNPNSGGS

SEQ ID NO: 212 - DNA, 24 bp, Artificial Sequence
  Description of Artificial Sequence: Synthetic oligonucleotide
gtgaacccaaatagcggaggctcc

SEQ ID NO: 213 - protein, 98 aa, Artificial Sequence; identical to SEQ ID NO: 11
  Description of Artificial Sequence: Synthetic polypeptide

SEQ ID NO: 214 - DNA, 294 bp, Artificial Sequence
  Description of Artificial Sequence: Synthetic polynucleotide
gcctccaccaagggaccttctgtgttcccactggctccctctagtaaatccacatctgggggaactgcagccctgggctgtctggtgaaggactacttcccagagcccgtcacagtgtcttggaacagtggcgctctgacttctggggtccacacctttcctgcagtgctgcagtcaagcgggctgtacagcctgtcctctgtggtcaccgtgccaagttcaagcctgggaacacagacttatatctgcaacgtgaatcacaagccatccaatacaaaagtcgacaagaaagtg

SEQ ID NO: 215 - protein, 110 aa, Artificial Sequence; identical to SEQ ID NO: 13
  Description of Artificial Sequence: Synthetic polypeptide

SEQ ID NO: 216 - DNA, 330 bp, Artificial Sequence; identical to SEQ ID NO: 30
  Description of Artificial Sequence: Synthetic polynucleotide

SEQ ID NO: 217 - protein, 106 aa, Artificial Sequence; identical to SEQ ID NO: 31
  Description of Artificial Sequence: Synthetic polypeptide

SEQ ID NO: 218 - DNA, 318 bp, Artificial Sequence; identical to SEQ ID NO: 32
  Description of Artificial Sequence: Synthetic polynucleotide

SEQ ID NO: 219 - protein, 448 aa, Artificial Sequence
  Description of Artificial Sequence: Synthetic polypeptide
EVQLVESGGGLVQPGGSLRLSCAASGFTFTDYTMDWVRQAPGKGLEWVADVNPNSGGSIYNQRFKGRFTLSVDRSKNTLYLQMNSLRAEDTAVYYCARNLGPSFYFDYWGQGTLVTVSSASTKGPSVFPLAPSSKSTSGGTAALGCLVKDYFPEPVTVSWNSGALTSGVHTFPAVLQSSGLYSLSSVVTVPSSSLGTQTYICNVNHKPSNTKVDKKVEPKSCDKTHTCPPCPAPELLGGPSVFLFPPKPKDTLMISRTPEVTCVVVDVSHEDPEVKFNWYVDGVEVHNAKTKPREEQYNSTYRVVSVLTVLHQDWLNGKEYKCKVSNKALPAPIEKTISKAKGQPREPQVYVYPPSRDELTKNQVSLTCLVKGFYPSDIAVEWESNGQPENNYKTTPPVLDSDGSFALVSKLTVDKSRWQQGNVFSCSVMHEALHNHYTQKSLSLSPG

SEQ ID NO: 220 - DNA, 1344 bp, Artificial Sequence
  Description of Artificial Sequence: Synthetic polynucleotide
gaagtgcagctggtcgaatctggaggaggactggtgcagccaggagggtccctgcgcctgtcttgcgccgctagtggcttcacttttaccgactacaccatggattgggtgcgacaggcacctggaaagggcctggagtgggtcgccgatgtgaacccaaatagcggaggctccatctacaaccagcggttcaagggccggttcaccctgtcagtggaccggagcaaaaacaccctgtatctgcagatgaatagcctgcgagccgaagatactgctgtgtactattgcgcccggaatctggggccctccttctactttgactattgggggcagggaactctggtcaccgtgagctccgcctccaccaagggaccttctgtgttcccactggctccctctagtaaatccacatctgggggaactgcagccctgggctgtctggtgaaggactacttcccagagcccgtcacagtgtcttggaacagtggcgctctgacttctggggtccacacctttcctgcagtgctgcagtcaagcgggctgtacagcctgtcctctgtggtcaccgtgccaagttcaagcctgggaacacagacttatatctgcaacgtgaatcacaagccatccaatacaaaagtcgacaagaaagtggaacccaagtcttgtgataaaacccatacatgccccccttgtcctgcaccagagctgctgggaggaccaagcgtgttcctgtttccacccaagcctaaagatacactgatgattagtaggaccccagaagtcacatgcgtggtcgtggacgtgagccacgaggaccccgaagtcaagtttaactggtacgtggacggcgtcgaggtgcataatgccaagactaaacccagggaggaacagtacaacagtacctatcgcgtcgtgtcagtcctgacagtgctgcatcaggattggctgaacgggaaagagtataagtgcaaagtgagcaataaggctctgcccgcacctatcgagaaaacaatttccaaggcaaaaggacagcctagagaaccacaggtgtacgtgtatcctccatcaagggatgagctgacaaagaaccaggtcagcctgacttgtctggtgaaaggattctatccctctgacattgctgtggagtgggaaagtaatggccagcctgagaacaattacaagaccacaccccctgtgctggactcagatggcagcttcgcgctggtgagcaagctgaccgtcgacaaatcccggtggcagcaggggaatgtgtttagttgttcagtcatgcacgaggcactgcacaaccattacacccagaagtcactgtcactgtcaccaggg

SEQ ID NO: 221 - protein, 119 aa, Artificial Sequence [sequence omitted]

SEQ ID NO: 222 - DNA, 357 bp, Artificial Sequence; identical to SEQ ID NO: 20
  Description of Artificial Sequence: Synthetic polynucleotide

SEQ ID NO: 223 - protein, 8 aa, Artificial Sequence
  Description of Artificial Sequence: Synthetic peptide
GFTFTDYT

SEQ ID NO: 224 - DNA, 24 bp, Artificial Sequence
  Description of Artificial Sequence: Synthetic oligonucleotide
ggcttcacttttaccgactacacc

SEQ ID NO: 225 - protein, 12 aa, Artificial Sequence
  Description of Artificial Sequence: Synthetic peptide
ARNLGPSFYFDY

SEQ ID NO: 226 - DNA, 36 bp, Artificial Sequence; identical to SEQ ID NO: 24
  Description of Artificial Sequence: Synthetic oligonucleotide

SEQ ID NO: 227 - protein, 8 aa, Artificial Sequence
  Description of Artificial Sequence: Synthetic peptide
VNPNSGGS

SEQ ID NO: 228 - DNA, 24 bp, Artificial Sequence
  Description of Artificial Sequence: Synthetic oligonucleotide
gtgaacccaaatagcggaggctcc

SEQ ID NO: 229 - protein, 98 aa, Artificial Sequence; identical to SEQ ID NO: 11
  Description of Artificial Sequence: Synthetic polypeptide

SEQ ID NO: 230 - DNA, 294 bp, Artificial Sequence; identical to SEQ ID NO: 214
  Description of Artificial Sequence: Synthetic polynucleotide

SEQ ID NO: 231 - protein, 110 aa, Artificial Sequence; identical to SEQ ID NO: 13
  Description of Artificial Sequence: Synthetic polypeptide

SEQ ID NO: 232 - DNA, 330 bp, Artificial Sequence; identical to SEQ ID NO: 30
  Description of Artificial Sequence: Synthetic polynucleotide

SEQ ID NO: 233 - protein, 106 aa, Artificial Sequence; identical to SEQ ID NO: 95
  Description of Artificial Sequence: Synthetic polypeptide

SEQ ID NO: 234 - DNA, 318 bp, Artificial Sequence
  Description of Artificial Sequence: Synthetic polynucleotide
ggacagcctagagaaccacaggtgtacgtgtatcctccatcaagggatgagctgacaaagaaccaggtcagcctgacttgtctggtgaaaggattctatccctctgacattgctgtggagtgggaaagtaatggccagcctgagaacaattacaagaccacaccccctgtgctggactcagatggcagcttcgcgctggtgagcaagctgaccgtcgacaaatcccggtggcagcaggggaatgtgtttagttgttcagtcatgcacgaggcactgcacaaccattacacccagaagtcactgtcactgtcaccaggg

SEQ ID NO: 235 - protein, 450 aa, Artificial Sequence; identical to SEQ ID NO: 125
  Description of Artificial Sequence: Synthetic polypeptide

SEQ ID NO: 236 - DNA, 1350 bp, Artificial Sequence
  Description of Artificial Sequence: Synthetic polynucleotide
gaggtgcagctggtggaaagcggaggaggactggtgcagccaggaggatctctgcgactgagttgcgccgcttcaggattcaacatcaaggacacctacattcactgggtgcgacaggctccaggaaaaggactggagtgggtggctcgaatctatcccactaatggatacacccggtatgccgactccgtgaaggggaggtttactattagcgccgatacatccaaaaacactgcttacctgcagatgaacagcctgcgagccgaagataccgctgtgtactattgcagtcgatggggaggagacggattctacgctatggattattggggacaggggaccctggtgacagtgagctccgcctctaccaagggccccagtgtgtttcccctggctccttctagtaaatccacctctggagggacagccgctctgggatgtctggtgaaggactatttccccgagcctgtgaccgtgagttggaactcaggcgccctgacaagcggagtgcacacttttcctgctgtgctgcagtcaagcgggctgtactccctgtcctctgtggtgacagtgccaagttcaagcctgggcacacagacttatatctgcaacgtgaatcataagccctcaaatacaaaagtggacaagaaagtggagcccaagagctgtgataagacccacacctgccctccctgtccagctccagaactgctgggaggacctagcgtgttcctgtttccccctaagccaaaagacactctgatgatttccaggactcccgaggtgacctgcgtggtggtggacgtgtctcacgaggaccccgaagtgaagttcaactggtacgtggatggcgtggaagtgcataatgctaagacaaaaccaagagaggaacagtacaactccacttatcgcgtcgtgagcgtgctgaccgtgctgcaccaggactggctgaacgggaaggagtataagtgcaaagtcagtaataaggccctgcctgctccaatcgaaaaaaccatctctaaggccaaaggccagccaagggagccccaggtgtacgtgtacccacccagcagagacgaactgaccaagaaccaggtgtccctgacatgtctggtgaaaggcttctatcctagtgatattgctgtggagtgggaatcaaatggacagccagagaacaattacaagaccacacctccagtgctggacagcgatggcagcttcgccctggtgtccaagctgacagtggataaatctcgatggcagcaggggaacgtgtttagttgttcagtgatgcatgaagccctgcacaatcattacactcagaagagcctgtccctgtctcccggcaaa

SEQ ID NO: 237 - protein, 120 aa, Artificial Sequence [sequence omitted]

SEQ ID NO: 238 - DNA, 360 bp, Artificial Sequence; identical to SEQ ID NO: 4
  Description of Artificial Sequence: Synthetic polynucleotide

SEQ ID NO: 239 - protein, 8 aa, Artificial Sequence
  Description of Artificial Sequence: Synthetic peptide
GFNIKDTY

SEQ ID NO: 240 - DNA, 24 bp, Artificial Sequence
  Description of Artificial Sequence: Synthetic oligonucleotide
ggattcaacatcaaggacacctac

SEQ ID NO: 241 - protein, 13 aa, Artificial Sequence
  Description of Artificial Sequence: Synthetic peptide
SRWGGDGFYAMDY

SEQ ID NO: 242 - DNA, 39 bp, Artificial Sequence; identical to SEQ ID NO: 8
  Description of Artificial Sequence: Synthetic oligonucleotide

SEQ ID NO: 243 - protein, 8 aa, Artificial Sequence
  Description of Artificial Sequence: Synthetic peptide
IYPTNGYT

SEQ ID NO: 244 - DNA, 24 bp, Artificial Sequence
  Description of Artificial Sequence: Synthetic oligonucleotide
atctatcccactaatggatacacc

SEQ ID NO: 245 - protein, 98 aa, Artificial Sequence; identical to SEQ ID NO: 11
  Description of Artificial Sequence: Synthetic polypeptide

SEQ ID NO: 246 - DNA, 294 bp, Artificial Sequence; identical to SEQ ID NO: 12
  Description of Artificial Sequence: Synthetic polynucleotide

SEQ ID NO: 247 - protein, 110 aa, Artificial Sequence; identical to SEQ ID NO: 13
  Description of Artificial Sequence: Synthetic polypeptide

SEQ ID NO: 248 - DNA, 330 bp, Artificial Sequence; identical to SEQ ID NO: 14
  Description of Artificial Sequence: Synthetic polynucleotide

SEQ ID NO: 249 - protein, 106 aa, Artificial Sequence; identical to SEQ ID NO: 95
  Description of Artificial Sequence: Synthetic polypeptide

SEQ ID NO: 250 - DNA, 318 bp, Artificial Sequence
  Description of Artificial Sequence: Synthetic polynucleotide
ggccagccaagggagccccaggtgtacgtgtacccacccagcagagacgaactgaccaagaaccaggtgtccctgacatgtctggtgaaaggcttctatcctagtgatattgctgtggagtgggaatcaaatggacagccagagaacaattacaagaccacacctccagtgctggacagcgatggcagcttcgccctggtgtccaagctgacagtggataaatctcgatggcagcaggggaacgtgtttagttgttcagtgatgcatgaagccctgcacaatcattacactcagaagagcctgtccctgtctcccggc

SEQ ID NO: 251 - protein, 232 aa, Artificial Sequence
  Description of Artificial Sequence: Synthetic polypeptide
EPKSSDKTHTCPPCPAPELLGGPSVFLFPPKPKDTLMISRTPEVTCVVVDVSHEDPEVKFNWYVDGVEVHNAKTKPREEQYNSTYRVVSVLTVLHQDWLNGKEYKCKVSNKALPAPIEKTISKAKGQPREPQVYVLPPSRDELTKNQVSLLCLVKGFYPSDIAVEWESNGQPENNYLTWPPVLDSDGSFFLYSKLTVDKSRWQQGNVFSCSVMHEALHNHYTQKSLSLSPGK

SEQ ID NO: 252 - DNA, 696 bp, Artificial Sequence
  Description of Artificial Sequence: Synthetic polynucleotide
gaacctaaaagcagcgacaagacccacacatgccccccttgtccagctccagaactgctgggaggaccaagcgtgttcctgtttccacccaagcccaaagatacactgatgatcagccgaactcccgaggtcacctgcgtggtcgtggacgtgtcccacgaggaccccgaagtcaagttcaactggtacgtggacggcgtcgaagtgcataatgcaaagactaaaccacgggaggaacagtacaactctacatatagagtcgtgagtgtcctgactgtgctgcatcaggattggctgaacggcaaagagtataagtgcaaagtgtctaataaggccctgcctgctccaatcgagaaaactattagtaaggcaaaagggcagcccagggaacctcaggtctacgtgctgcctccaagtcgcgacgagctgaccaagaaccaggtctcactgctgtgtctggtgaaaggattctatccttccgatattgccgtggagtgggaatctaatggccagccagagaacaattacctgacctggccccctgtgctggacagcgatgggtccttctttctgtattcaaagctgacagtggacaaaagcagatggcagcagggaaacgtctttagctgttccgtgatgcacgaagccctgcacaatcattacacccagaagtctctgagtctgtcacctggcaaa

SEQ ID NO: 253 - protein, 110 aa, Artificial Sequence; identical to SEQ ID NO: 13
  Description of Artificial Sequence: Synthetic polypeptide

SEQ ID NO: 254 - DNA, 330 bp, Artificial Sequence
  Description of Artificial Sequence: Synthetic polynucleotide
gctccagaactgctgggaggaccaagcgtgttcctgtttccacccaagcccaaagatacactgatgatcagccgaactcccgaggtcacctgcgtggtcgtggacgtgtcccacgaggaccccgaagtcaagttcaactggtacgtggacggcgtcgaagtgcataatgcaaagactaaaccacgggaggaacagtacaactctacatatagagtcgtgagtgtcctgactgtgctgcatcaggattggctgaacggcaaagagtataagtgcaaagtgtctaataaggccctgcctgctccaatcgagaaaactattagtaaggcaaaa

SEQ ID NO: 255 - protein, 106 aa, Artificial Sequence; identical to SEQ ID NO: 31
  Description of Artificial Sequence: Synthetic polypeptide

SEQ ID NO: 256 - DNA, 318 bp, Artificial Sequence
  Description of Artificial Sequence: Synthetic polynucleotide
gggcagcccagggaacctcaggtctacgtgctgcctccaagtcgcgacgagctgaccaagaaccaggtctcactgctgtgtctggtgaaaggattctatccttccgatattgccgtggagtgggaatctaatggccagccagagaacaattacctgacctggccccctgtgctggacagcgatgggtccttctttctgtattcaaagctgacagtggacaaaagcagatggcagcagggaaacgtctttagctgttccgtgatgcacgaagccctgcacaatcattacacccagaagtctctgagtctgtcacctggc

SEQ ID NO: 257 - protein, 475 aa, Artificial Sequence
  Description of Artificial Sequence: Synthetic polypeptide
DIQMTQSPSSLSASVGDRVTITCKASQDVSIGVAWYQQKPGKAPKLLIYSASYRYTGVPSRFSGSGSGTDFTLTISSLQPEDFATYYCQQYYIYPYTFGQGTKVEIKGGGGSGGGGSGGGGSEVQLVESGGGLVQPGGSLRLSCAASGFTFTDYTMDWVRQAPGKGLEWVADVNPNSGGSIYNQRFKGRFTLSVDRSKNTLYLQMNSLRAEDTAVYYCARNLGPSFYFDYWGQGTLVTVSSAAEPKSSDKTHTCPPCPAPELLGGPSVFLFPPKPKDTLMISRTPEVTCVVVDVSHEDPEVKFNWYVDGVEVHNAKTKPREEQYNSTYRVVSVLTVLHQDWLNGKEYKCKVSNKALPAPIEKTISKAKGQPREPQVYVYPPSRDELTKNQVSLTCLVKGFYPSDIAVEWESNGQPENNYKTTPPVLDSDGSFALVSKLTVDKSRWQQGNVFSCSVMHEALHNHYTQKSLSLSPGK

SEQ ID NO: 258 - DNA, 1425 bp, Artificial Sequence
  Description of Artificial Sequence: Synthetic polynucleotide
gacattcagatgacccagagccctagctccctgagtgcctcagtcggggacagggtgactatcacctgcaaggcttcacaggatgtcagcattggcgtggcatggtaccagcagaagccagggaaagcacccaagctgctgatctatagcgcctcctacaggtatacaggcgtgccatcccgcttctctggcagtgggtcaggaactgactttacactgactatttctagtctgcagcccgaagatttcgccacatactattgccagcagtactatatctacccttatacttttggccaggggaccaaagtggagattaagggcggaggaggctccggaggaggagggtctggaggaggaggaagtgaggtccagctggtggaatctggaggaggactggtgcagccaggagggtccctgaggctgtcttgtgccgctagtggcttcacctttacagactacacaatggattgggtgcgccaggcaccaggaaagggactggaatgggtcgctgatgtgaaccctaatagcggaggctccatctacaaccagcggttcaaaggacggttcaccctgtcagtggaccggagcaagaacaccctgtatctgcagatgaacagcctgagagccgaggatactgctgtgtactattgcgccaggaatctgggcccaagcttctactttgactattgggggcagggaacactggtcactgtgtcaagcgcagccgaacccaaatcctctgataagactcacacctgcccaccttgtccagctccagagctgctgggaggacctagcgtgttcctgtttccacccaagccaaaagacactctgatgatttctagaacccctgaagtgacatgtgtggtcgtggacgtcagtcacgaggaccccgaagtcaaattcaactggtacgtggatggcgtcgaggtgcataatgccaagaccaaaccccgagaggaacagtacaactcaacctatcgggtcgtgagcgtcctgacagtgctgcatcaggactggctgaacggcaaggagtataagtgcaaagtgagcaacaaggctctgcctgcaccaatcgagaagaccatttccaaggctaaagggcagccccgcgaacctcaggtctacgtgtatcctccaagccgagatgagctgacaaaaaaccaggtctccctgacttgtctggtgaagggattttacccaagtgacatcgcagtggagtgggaatcaaatggccagcccgaaaacaattataagaccacaccccctgtgctggactctgatgggagtttcgcactggtctccaaactgaccgtggacaagtctcggtggcagcagggaaacgtctttagctgttccgtgatgcacgaggccctgcacaatcattacacacagaaatctctgagtctgtcacctggcaag

SEQ ID NO: 259 - protein, 107 aa, Artificial Sequence [sequence omitted]

SEQ ID NO: 260 - DNA, 321 bp, Artificial Sequence
  Description of Artificial Sequence: Synthetic polynucleotide
gacattcagatgacccagagccctagctccctgagtgcctcagtcggggacagggtgactatcacctgcaaggcttcacaggatgtcagcattggcgtggcatggtaccagcagaagccagggaaagcacccaagctgctgatctatagcgcctcctacaggtatacaggcgtgccatcccgcttctctggcagtgggtcaggaactgactttacactgactatttctagtctgcagcccgaagatttcgccacatactattgccagcagtactatatctacccttatacttttggccaggggaccaaagtggagattaag

SEQ ID NO: 261 - protein, 6 aa, Artificial Sequence
  Description of Artificial Sequence: Synthetic peptide
QDVSIG

SEQ ID NO: 262 - DNA, 18 bp, Artificial Sequence
  Description of Artificial Sequence: Synthetic oligonucleotide
caggatgtcagcattggc

SEQ ID NO: 263 - protein, 9 aa, Artificial Sequence
  Description of Artificial Sequence: Synthetic peptide
QQYYIYPYT

SEQ ID NO: 264 - DNA, 27 bp, Artificial Sequence
  Description of Artificial Sequence: Synthetic oligonucleotide
cagcagtactatatctacccttatact

SEQ ID NO: 265 - protein, 3 aa, Artificial Sequence
  Description of Artificial Sequence: Synthetic peptide
SAS

SEQ ID NO: 266 - DNA, 9 bp, Artificial Sequence
  Description of Artificial Sequence: Synthetic oligonucleotide
agcgcctcc

SEQ ID NO: 267 - protein, 119 aa, Artificial Sequence [sequence omitted]

SEQ ID NO: 268 - DNA, 357 bp, Artificial Sequence
  Description of Artificial Sequence: Synthetic polynucleotide
gaggtccagctggtggaatctggaggaggactggtgcagccaggagggtccctgaggctgtcttgtgccgctagtggcttcacctttacagactacacaatggattgggtgcgccaggcaccaggaaagggactggaatgggtcgctgatgtgaaccctaatagcggaggctccatctacaaccagcggttcaaaggacggttcaccctgtcagtggaccggagcaagaacaccctgtatctgcagatgaacagcctgagagccgaggatactgctgtgtactattgcgccaggaatctgggcccaagcttctactttgactattgggggcagggaacactggtcactgtgtcaagc

SEQ ID NO: 269 - protein, 8 aa, Artificial Sequence
  Description of Artificial Sequence: Synthetic peptide
GFTFTDYT

SEQ ID NO: 270 - DNA, 24 bp, Artificial Sequence
  Description of Artificial Sequence: Synthetic oligonucleotide
ggcttcacctttacagactacaca

SEQ ID NO: 271 - protein, 12 aa, Artificial Sequence
  Description of Artificial Sequence: Synthetic peptide
ARNLGPSFYFDY

SEQ ID NO: 272 - DNA, 36 bp, Artificial Sequence
  Description of Artificial Sequence: Synthetic oligonucleotide
gccaggaatctgggcccaagcttctactttgactat

SEQ ID NO: 273 - protein, 8 aa, Artificial Sequence
  Description of Artificial Sequence: Synthetic peptide
VNPNSGGS

SEQ ID NO: 274 - DNA, 24 bp, Artificial Sequence
  Description of Artificial Sequence: Synthetic oligonucleotide
gtgaaccctaatagcggaggctcc

SEQ ID NO: 275 - protein, 110 aa, Artificial Sequence; identical to SEQ ID NO: 13
  Description of Artificial Sequence: Synthetic polypeptide

SEQ ID NO: 276 - DNA, 330 bp, Artificial Sequence
  Description of Artificial Sequence: Synthetic polynucleotide
gctccagagctgctgggaggacctagcgtgttcctgtttccacccaagccaaaagacactctgatgatttctagaacccctgaagtgacatgtgtggtcgtggacgtcagtcacgaggaccccgaagtcaaattcaactggtacgtggatggcgtcgaggtgcataatgccaagaccaaaccccgagaggaacagtacaactcaacctatcgggtcgtgagcgtcctgacagtgctgcatcaggactggctgaacggcaaggagtataagtgcaaagtgagcaacaaggctctgcctgcaccaatcgagaagaccatttccaaggctaaa

SEQ ID NO: 277 - protein, 106 aa, Artificial Sequence; identical to SEQ ID NO: 95
  Description of Artificial Sequence: Synthetic polypeptide

SEQ ID NO: 278 - DNA, 318 bp, Artificial Sequence
  Description of Artificial Sequence: Synthetic polynucleotide
gggcagccccgcgaacctcaggtctacgtgtatcctccaagccgagatgagctgacaaaaaaccaggtctccctgacttgtctggtgaagggattttacccaagtgacatcgcagtggagtgggaatcaaatggccagcccgaaaacaattataagaccacaccccctgtgctggactctgatgggagtttcgcactggtctccaaactgaccgtggacaagtctcggtggcagcagggaaacgtctttagctgttccgtgatgcacgaggccctgcacaatcattacacacagaaatctctgagtctgtcacctggc

SEQ ID NO: 279 - protein, 450 aa, Artificial Sequence
  Description of Artificial Sequence: Synthetic polypeptide
EVQLVESGGGLVQPGGSLRLSCAASGFNIKDTYIHWVRQAPGKGLEWVARIYPTNGYTRYADSVKGRFTISADTSKNTAYLQMNSLRAEDTAVYYCSRWGGDGFYAMDYWGQGTLVTVSSASTKGPSVFPLAPSSKSTSGGTAALGCLVKDYFPEPVTVSWNSGALTSGVHTFPAVLQSSGLYSLSSVVTVPSSSLGTQTYICNVNHKPSNTKVDKKVEPKSCDKTHTCPPCPAPELLGGPSVFLFPPKPKDTLMISRTPEVTCVVVDVSHEDPEVKFNWYVDGVEVHNAKTKPREEQYNSTYRVVSVLTVLHQDWLNGKEYKCKVSNKALPAPIEKTISKAKGQPREPQVYVLPPSRDELTKNQVSLLCLVKGFYPSDIAVEWESNGQPENNYLTWPPVLDSDGSFFLYSKLTVDKSRWQQGNVFSCSVMHEALHNHYTQKSLSLSPGK

SEQ ID NO: 280 - DNA, 1350 bp, Artificial Sequence
  Description of Artificial Sequence: Synthetic polynucleotide
gaggtgcagctggtggaaagcggaggaggactggtgcagccaggaggatctctgcgactgagttgcgccgcttcaggattcaacatcaaggacacctacattcactgggtgcgacaggctccaggaaaaggactggagtgggtggctcgaatctatcccactaatggatacacccggtatgccgactccgtgaaggggaggtttactattagcgccgatacatccaaaaacactgcttacctgcagatgaacagcctgcgagccgaagataccgctgtgtactattgcagtcgatggggaggagacggattctacgctatggattattggggacaggggaccctggtgacagtgagctccgcctctaccaagggccccagtgtgtttcccctggctccttctagtaaatccacctctggagggacagccgctctgggatgtctggtgaaggactatttccccgagcctgtgaccgtgagttggaactcaggcgccctgacaagcggagtgcacacttttcctgctgtgctgcagtcaagcgggctgtactccctgtcctctgtggtgacagtgccaagttcaagcctgggcacacagacttatatctgcaacgtgaatcataagccctcaaatacaaaagtggacaagaaagtggagcccaagagctgtgataagacccacacctgccctccctgtccagctccagaactgctgggaggacctagcgtgttcctgtttccccctaagccaaaagacactctgatgatttccaggactcccgaggtgacctgcgtggtggtggacgtgtctcacgaggaccccgaagtgaagttcaactggtacgtggatggcgtggaagtgcataatgctaagacaaaaccaagagaggaacagtacaactccacttatcgcgtcgtgagcgtgctgaccgtgctgcaccaggactggctgaacgggaaggagtataagtgcaaagtcagtaataaggccctgcctgctccaatcgaaaaaaccatctctaaggccaaaggccagccaagggagccccaggtgtacgtgctgccacccagcagagacgaactgaccaagaaccaggtgtccctgctgtgtctggtgaaaggcttctatcctagtgatattgctgtggagtgggaatcaaatggacagccagagaacaattacctgacctggcctccagtgctggacagcgatggcagcttcttcctgtattccaagctgacagtggataaatctcgatggcagcaggggaacgtgtttagttgttcagtgatgcatgaagccctgcacaatcattacactcagaagagcctgtccctgtctcccggcaaa

SEQ ID NO: 281 - protein, 120 aa, Artificial Sequence [sequence omitted]

SEQ ID NO: 282 - DNA, 360 bp, Artificial Sequence; identical to SEQ ID NO: 4
  Description of Artificial Sequence: Synthetic polynucleotide

SEQ ID NO: 283 - protein, 8 aa, Artificial Sequence
  Description of Artificial Sequence: Synthetic peptide
GFNIKDTY

SEQ ID NO: 284 - DNA, 24 bp, Artificial Sequence
  Description of Artificial Sequence: Synthetic oligonucleotide
ggattcaacatcaaggacacctac

SEQ ID NO: 285 - protein, 13 aa, Artificial Sequence
  Description of Artificial Sequence: Synthetic peptide
SRWGGDGFYAMDY

SEQ ID NO: 286 - DNA, 39 bp, Artificial Sequence; identical to SEQ ID NO: 8
  Description of Artificial Sequence: Synthetic oligonucleotide

SEQ ID NO: 287 - protein, 8 aa, Artificial Sequence
  Description of Artificial Sequence: Synthetic peptide
IYPTNGYT

SEQ ID NO: 288 - DNA, 24 bp, Artificial Sequence
  Description of Artificial Sequence: Synthetic oligonucleotide
atctatcccactaatggatacacc

SEQ ID NO: 289 - protein, 98 aa, Artificial Sequence; identical to SEQ ID NO: 11
  Description of Artificial Sequence: Synthetic polypeptide

SEQ ID NO: 290 - DNA, 294 bp, Artificial Sequence; identical to SEQ ID NO: 12
  Description of Artificial Sequence: Synthetic polynucleotide

SEQ ID NO: 291 - protein, 110 aa, Artificial Sequence; identical to SEQ ID NO: 13
  Description of Artificial Sequence: Synthetic polypeptide

SEQ ID NO: 292 - DNA, 330 bp, Artificial Sequence; identical to SEQ ID NO: 14
  Description of Artificial Sequence: Synthetic polynucleotide

SEQ ID NO: 293 - protein, 106 aa, Artificial Sequence; identical to SEQ ID NO: 31
  Description of Artificial Sequence: Synthetic polypeptide

SEQ ID NO: 294 - DNA, 318 bp, Artificial Sequence
  Description of Artificial Sequence: Synthetic polynucleotide
ggccagccaagggagccccaggtgtacgtgctgccacccagcagagacgaactgaccaagaaccaggtgtccctgctgtgtctggtgaaaggcttctatcctagtgatattgctgtggagtgggaatcaaatggacagccagagaacaattacctgacctggcctccagtgctggacagcgatggcagcttcttcctgtattccaagctgacagtggataaatctcgatggcagcaggggaacgtgtttagttgttcagtgatgcatgaagccctgcacaatcattacactcagaagagcctgtccctgtctcccggc

SEQ ID NO: 295 - protein, 480 aa, Artificial Sequence
  Description of Artificial Sequence: Synthetic polypeptide
DIQMTQSPSSLSASVGDRVTITCRASQDVNTAVAWYQQKPGKAPKLLIYSASFLYSGVPSRFSGSRSGTDFTLTISSLQPEDFATYYCQQHYTTPPTFGQGTKVEIKGGSGGGSGGGSGGGSGGGSGEVQLVESGGGLVQPGGSLRLSCAASGFNIKDTYIHWVRQAPGKGLEWVARIYPTNGYTRYADSVKGRFTISADTSKNTAYLQMNSLRAEDTAVYYCSRWGGDGFYAMDYWGQGTLVTVSSAAEPKSSDKTHTCPPCPAPELLGGPSVFLFPPKPKDTLMISRTPEVTCVVVDVSHEDPEVKFNWYVDGVEVHNAKTKPREEQYNSTYRVVSVLTVLHQDWLNGKEYKCKVSNKALPAPIEKTISKAKGQPREPQVYVLPPSRDELTKNQVSLLCLVKGFYPSDIAVEWESNGQPENNYLTWPPVLDSDGSFFLYSKLTVDKSRWQQGNVFSCSVMHEALHNHYTQKSLSLSPG

SEQ ID NO: 296 - DNA, 1440 bp, Artificial Sequence
  Description of Artificial Sequence: Synthetic polynucleotide
gacattcagatgacacagagccccagctccctgagtgcttcagtcggcgacagggtgactatcacctgccgcgcatcccaggatgtcaacaccgctgtggcatggtaccagcagaagcctggaaaagccccaaagctgctgatctacagcgcttccttcctgtattctggcgtgccaagtcggttttctggaagtagatcaggcactgacttcacactgactatctctagtctgcagcccgaagattttgccacctactattgccagcagcactataccacaccccctacattcggacagggcactaaagtggagattaagggcgggtcaggcggagggagcggaggagggtccggaggagggtctggaggagggagtggagaggtccagctggtggaatctggaggaggactggtgcagcctggaggctcactgcgactgagctgtgccgcttccggctttaacatcaaagacacatacattcattgggtcaggcaggcaccagggaagggactggaatgggtggcccgcatctatcccacaaatgggtacactcgatatgccgacagcgtgaaaggacggtttaccatttctgctgataccagtaagaacacagcatacctgcagatgaacagcctgcgcgcagaggatacagccgtgtactattgcagtcgatgggggggagacggcttctacgccatggattattggggccaggggactctggtcaccgtgtcaagcgcagccgaacctaaatcctctgacaagacccacacatgcccaccctgtcctgctccagagctgctgggaggaccatccgtgttcctgtttcctccaaagcctaaagatacactgatgattagccgcactcccgaagtcacctgtgtggtcgtggacgtgtcccacgaggaccccgaagtcaagttcaactggtacgtggacggcgtcgaggtgcataatgccaagactaaaccaagagaggaacagtacaattcaacctatagggtcgtgagcgtcctgacagtgctgcatcaggattggctgaacggcaaggagtataagtgcaaagtgtctaacaaggccctgcccgctcctatcgagaagactattagcaaggcaaaagggcagccacgggaaccccaggtctacgtgctgccccctagcagagacgagctgaccaaaaaccaggtctccctgctgtgtctggtgaagggcttttatcctagtgatatcgctgtggagtgggaatcaaatgggcagccagaaaacaattacctgacatggccacccgtgctggacagcgatgggtccttctttctgtattccaaactgactgtggacaagtctagatggcagcagggaaacgtcttcagctgttccgtgatgcacgaggccctgcacaatcattacacccagaagtctctgagtctgtcacccggc

SEQ ID NO: 297 - protein, 107 aa, Artificial Sequence [sequence omitted]

SEQ ID NO: 298 - DNA, 321 bp, Artificial Sequence
  Description of Artificial Sequence: Synthetic polynucleotide
gacattcagatgacacagagccccagctccctgagtgcttcagtcggcgacagggtgactatcacctgccgcgcatcccaggatgtcaacaccgctgtggcatggtaccagcagaagcctggaaaagccccaaagctgctgatctacagcgcttccttcctgtattctggcgtgccaagtcggttttctggaagtagatcaggcactgacttcacactgactatctctagtctgcagcccgaagattttgccacctactattgccagcagcactataccacaccccctacattcggacagggcactaaagtggagattaag

SEQ ID NO: 299 - protein, 6 aa, Artificial Sequence
  Description of Artificial Sequence: Synthetic peptide
QDVNTA

SEQ ID NO: 300 - DNA, 18 bp, Artificial Sequence
  Description of Artificial Sequence: Synthetic oligonucleotide
caggatgtcaacaccgct

SEQ ID NO: 301 - protein, 9 aa, Artificial Sequence
  Description of Artificial Sequence: Synthetic peptide
QQHYTTPPT

SEQ ID NO: 302 - DNA, 27 bp, Artificial Sequence
  Description of Artificial Sequence: Synthetic oligonucleotide
cagcagcactataccacaccccctaca

SEQ ID NO: 303 - protein, 3 aa, Artificial Sequence
  Description of Artificial Sequence: Synthetic peptide
SAS

SEQ ID NO: 304 - DNA, 9 bp, Artificial Sequence
  Description of Artificial Sequence: Synthetic oligonucleotide
agcgcttcc

SEQ ID NO: 305 - protein, 120 aa, Artificial Sequence [sequence omitted]

SEQ ID NO: 306 - DNA, 360 bp, Artificial Sequence
  Description of Artificial Sequence: Synthetic polynucleotide
gaggtccagctggtggaatctggaggaggactggtgcagcctggaggctcactgcgactgagctgtgccgcttccggctttaacatcaaagacacatacattcattgggtcaggcaggcaccagggaagggactggaatgggtggcccgcatctatcccacaaatgggtacactcgatatgccgacagcgtgaaaggacggtttaccatttctgctgataccagtaagaacacagcatacctgcagatgaacagcctgcgcgcagaggatacagccgtgtactattgcagtcgatgggggggagacggcttctacgccatggattattggggccaggggactctggtcaccgtgtcaagc

SEQ ID NO: 307 - protein, 8 aa, Artificial Sequence
  Description of Artificial Sequence: Synthetic peptide
GFNIKDTY

SEQ ID NO: 308 - DNA, 24 bp, Artificial Sequence
  Description of Artificial Sequence: Synthetic oligonucleotide
ggctttaacatcaaagacacatac

SEQ ID NO: 309 - protein, 13 aa, Artificial Sequence
  Description of Artificial Sequence: Synthetic peptide
SRWGGDGFYAMDY

SEQ ID NO: 310 - DNA, 39 bp, Artificial Sequence
  Description of Artificial Sequence: Synthetic oligonucleotide
agtcgatgggggggagacggcttctacgccatggattat

SEQ ID NO: 311 - protein, 8 aa, Artificial Sequence
  Description of Artificial Sequence: Synthetic peptide
IYPTNGYT

SEQ ID NO: 312 - DNA, 24 bp, Artificial Sequence
  Description of Artificial Sequence: Synthetic oligonucleotide
atctatcccacaaatgggtacact

SEQ ID NO: 313 - protein, 110 aa, Artificial Sequence; identical to SEQ ID NO: 13
  Description of Artificial Sequence: Synthetic polypeptide

SEQ ID NO: 314 - DNA, 330 bp, Artificial Sequence
  Description of Artificial Sequence: Synthetic polynucleotide
gctccagagctgctgggaggaccatccgtgttcctgtttcctccaaagcctaaagatacactgatgattagccgcactcccgaagtcacctgtgtggtcgtggacgtgtcccacgaggaccccgaagtcaagttcaactggtacgtggacggcgtcgaggtgcataatgccaagactaaaccaagagaggaacagtacaattcaacctatagggtcgtgagcgtcctgacagtgctgcatcaggattggctgaacggcaaggagtataagtgcaaagtgtctaacaaggccctgcccgctcctatcgagaagactattagcaaggcaaaa

SEQ ID NO: 315 - protein, 106 aa, Artificial Sequence; identical to SEQ ID NO: 31
  Description of Artificial Sequence: Synthetic polypeptide

SEQ ID NO: 316 - DNA, 318 bp, Artificial Sequence
  Description of Artificial Sequence: Synthetic polynucleotide
gggcagccacgggaaccccaggtctacgtgctgccccctagcagagacgagctgaccaaaaaccaggtctccctgctgtgtctggtgaagggcttttatcctagtgatatcgctgtggagtgggaatcaaatgggcagccagaaaacaattacctgacatggccacccgtgctggacagcgatgggtccttctttctgtattccaaactgactgtggacaagtctagatggcagcagggaaacgtcttcagctgttccgtgatgcacgaggccctgcacaatcattacacccagaagtctctgagtctgtcacccggc

SEQ ID NO: 317 - protein, 214 aa, Artificial Sequence; identical to SEQ ID NO: 191
  Description of Artificial Sequence: Synthetic polypeptide

SEQ ID NO: 318 - DNA, 642 bp, Artificial Sequence
  Description of Artificial Sequence: Synthetic polynucleotide
gacatccagatgacccagtctccatcctccctgtctgcatctgtaggagacagagtcaccatcacttgccgggcaagtcaggacgttaacaccgctgtagcttggtatcagcagaaaccagggaaagcccctaagctcctgatctattctgcatcctttttgtacagtggggtcccatcaaggttcagtggcagtcgatctgggacagatttcactctcaccatcagcagtctgcaacctgaagattttgcaacttactactgtcaacagcattacactaccccacccactttcggccaagggaccaaagtggagatcaaacgaactgtggctgcaccatctgtcttcatcttcccgccatctgatgagcagttgaaatctggaactgcctctgttgtgtgcctgctgaataacttctatcccagagaggccaaagtacagtggaaggtggataacgccctccaatcgggtaactcccaagagagtgtcacagagcaggacagcaaggacagcacctacagcctcagcagcaccctgacgctgagcaaagcagactacgagaaacacaaagtctacgcctgcgaagtcacccatcagggcctgagctcgcccgtcacaaagagcttcaacaggggagagtgt

SEQ ID NO: 319 - protein, 107 aa, Artificial Sequence [sequence omitted]

SEQ ID NO: 320 - DNA, 321 bp, Artificial Sequence; identical to SEQ ID NO: 150
  Description of Artificial Sequence: Synthetic polynucleotide

SEQ ID NO: 321 - protein, 6 aa, Artificial Sequence
  Description of Artificial Sequence: Synthetic peptide
QDVNTA

SEQ ID NO: 322 - DNA, 18 bp, Artificial Sequence
  Description of Artificial Sequence: Synthetic oligonucleotide
caggacgttaacaccgct

SEQ ID NO: 323 - protein, 9 aa, Artificial Sequence
  Description of Artificial Sequence: Synthetic peptide
QQHYTTPPT

SEQ ID NO: 324 - DNA, 27 bp, Artificial Sequence
  Description of Artificial Sequence: Synthetic oligonucleotide
caacagcattacactaccccacccact

SEQ ID NO: 325 - protein, 3 aa, Artificial Sequence
  Description of Artificial Sequence: Synthetic peptide
SAS

SEQ ID NO: 326 - DNA, 9 bp, Artificial Sequence
  Description of Artificial Sequence: Synthetic oligonucleotide
tctgcatcc

SEQ ID NO: 327 - protein, 107 aa, Artificial Sequence [sequence omitted]

SEQ ID NO: 328 - DNA, 321 bp, Artificial Sequence
  Description of Artificial Sequence: Synthetic polynucleotide
cgaactgtggctgcaccatctgtcttcatcttcccgccatctgatgagcagttgaaatctggaactgcctctgttgtgtgcctgctgaataacttctatcccagagaggccaaagtacagtggaaggtggataacgccctccaatcgggtaactcccaagagagtgtcacagagcaggacagcaaggacagcacctacagcctcagcagcaccctgacgctgagcaaagcagactacgagaaacacaaagtctacgcctgcgaagtcacccatcagggcctgagctcgcccgtcacaaagagcttcaacaggggagagtgt

SEQ ID NO: 329 - protein, 231 aa, Artificial Sequence
  Description of Artificial Sequence: Synthetic polypeptide
EPKSSDKTHTCPPCPAPELLGGPSVFLFPPKPKDTLMISRTPEVTCVVVDVSHEDPEVKFNWYVDGVEVHNAKTKPREEQYNSTYRVVSVLTVLHQDWLNGKEYKCKVSNKALPAPIEKTISKAKGQPREPQVYVLPPSRDELTKNQVSLLCLVKGFYPSDIAVEWESNGQPENNYLTWPPVLDSDGSFFLYSKLTVDKSRWQQGNVFSCSVMHEALHNHYTQKSLSLSPG

SEQ ID NO: 330 - DNA, 693 bp, Artificial Sequence
  Description of Artificial Sequence: Synthetic polynucleotide
gaacctaaatccagcgacaagacccacacatgccccccttgtccagctccagaactgctgggaggaccaagcgtgttcctgtttccacccaagcccaaagatacactgatgatcagccgaactcccgaggtcacctgcgtggtcgtggacgtgtcccacgaggaccccgaagtcaagttcaactggtacgtggacggcgtcgaagtgcataatgcaaagactaaaccacgggaggaacagtacaactctacatatagagtcgtgagtgtcctgactgtgctgcatcaggattggctgaacggcaaagagtataagtgcaaagtgtctaataaggccctgcctgctccaatcgagaaaactattagtaaggcaaaagggcagcccagggaacctcaggtctacgtgctgcctccaagtcgcgacgagctgaccaagaaccaggtctcactgctgtgtctggtgaaaggattctatccttccgatattgccgtggagtgggaatctaatggccagccagagaacaattacctgacctggccccctgtgctggacagcgatgggtccttctttctgtattcaaagctgacagtggacaaaagcagatggcagcagggaaacgtctttagctgttccgtgatgcacgaagccctgcacaatcattacacccagaagtctctgagtctgtcacctggc

SEQ ID NO: 331 - protein, 110 aa, Artificial Sequence; identical to SEQ ID NO: 13
  Description of Artificial Sequence: Synthetic polypeptide

SEQ ID NO: 332 - DNA, 330 bp, Artificial Sequence; identical to SEQ ID NO: 254
  Description of Artificial Sequence: Synthetic polynucleotide

SEQ ID NO: 333 - protein, 106 aa, Artificial Sequence; identical to SEQ ID NO: 31
  Description of Artificial Sequence: Synthetic polypeptide

SEQ ID NO: 334 - DNA, 318 bp, Artificial Sequence; identical to SEQ ID NO: 256
  Description of Artificial Sequence: Synthetic polynucleotide

SEQ ID NO: 335 - protein, 8 aa, Artificial Sequence
  Description of Artificial Sequence: Synthetic peptide
VNPNSGGS

SEQ ID NO: 336 - protein, 12 aa, Artificial Sequence
  Description of Artificial Sequence: Synthetic peptide
ARNLGPSFYFDY

SEQ ID NO: 337 - protein, 8 aa, Artificial Sequence
  Description of Artificial Sequence: Synthetic peptide
GFTFTDYT

SEQ ID NO: 338 - protein, 3 aa, Artificial Sequence
  Description of Artificial Sequence: Synthetic peptide
SAS

SEQ ID NO: 339 - protein, 9 aa, Artificial Sequence
  Description of Artificial Sequence: Synthetic peptide
QQYYIYPYT

SEQ ID NO: 340 - protein, 6 aa, Artificial Sequence
  Description of Artificial Sequence: Synthetic peptide
QDVSIG

SEQ ID NO: 341 - protein, 8 aa, Artificial Sequence
  Description of Artificial Sequence: Synthetic peptide
IYPTNGYT

SEQ ID NO: 342 - protein, 13 aa, Artificial Sequence
  Description of Artificial Sequence: Synthetic peptide
SRWGGDGFYAMDY

SEQ ID NO: 343 - protein, 8 aa, Artificial Sequence
  Description of Artificial Sequence: Synthetic peptide
GFNIKDTY

SEQ ID NO: 344 - protein, 3 aa, Artificial Sequence
  Description of Artificial Sequence: Synthetic peptide
SAS

SEQ ID NO: 345 - protein, 9 aa, Artificial Sequence
  Description of Artificial Sequence: Synthetic peptide
QQHYTTPPT

SEQ ID NO: 346 - protein, 6 aa, Artificial Sequence
  Description of Artificial Sequence: Synthetic peptide
QDVNTA

SEQ ID NO: 347 - protein, 9 aa, Artificial Sequence
  Description of Artificial Sequence: Synthetic peptide
QQYYIYPAT

SEQ ID NO: 348 - protein, 8 aa, Artificial Sequence
  Description of Artificial Sequence: Synthetic peptide
GFTFADYT

SEQ ID NO: 349 - protein, 607 aa, Homo sapiens
TQVCTGTDMKLRLPASPETHLDMLRHLYQGCQVVQGNLELTYLPTNASLSFLQDIQEVQGYVLIAHNQVRQVPLQRLRIVRGTQLFEDNYALAVLDNGDPLNNTTPVTGASPGGLRELQLRSLTEILKGGVLIQRNPQLCYQDTILWKDIFHKNNQLALTLIDTNRSRACHPCSPMCKGSRCWGESSEDCQSLTRTVCAGGCARCKGPLPTDCCHEQCAAGCTGPKHSDCLACLHFNHSGICELHCPALVTYNTDTFESMPNPEGRYTFGASCVTACPYNYLSTDVGSCTLVCPLHNQEVTAEDGTQRCEKCSKPCARVCYGLGMEHLREVRAVTSANIQEFAGCKKIFGSLAFLPESFDGDPASNTAPLQPEQLQVFETLEEITGYLYISAWPDSLPDLSVFQNLQVIRGRILHNGAYSLTLQGLGISWLGLRSLRELGSGLALIHHNTHLCFVHTVPWDQLFRNPHQALLHTANRPEDECVGEGLACHQLCARGHCWGPGPTQCVNCSQFLRGQECVEECRVLQGLPREYVNARHCLPCHPECQPQNGSVTCFGPEADQCVACAHYKDPPFCVARCPSGVKPDLSYMPIWKFPDEEGACQPCPIN

SEQ ID NO: 350 - protein, 217 aa, Homo sapiens
APELLGGPSVFLFPPKPKDTLMISRTPEVTCVVVDVSHEDPEVKFNWYVDGVEVHNAKTKPREEQYNSTYRVVSVLTVLHQDWLNGKEYKCKVSNKALPAPIEKTISKAKGQPREPQVYTLPPSRDELTKNQVSLTCLVKGFYPSDIAVEWESNGQPENNYKTTPPVLDSDGSFFLYSKLTVDKSRWQQGNVFSCSVMHEALHNHYTQKSLSLSPGK